European Patent Application EP 4 234 689 A2, published August 30, 2023. Title: SPLIT INTEINS WITH EXCEPTIONAL SPLICING ACTIVITY. Applicant: THE TRUSTEES OF PRINCETON UNIVERSITY. The sequence listing filed with the application follows.

SEQUENCE LISTING (499 sequences)

SEQ ID NO: 1 - protein, 92 aa, synthetic construct
  source 1..92: note = synthetic polypeptide
CLSYDTEILTVEYGFLPIGKIVEERIECTVYTVDKNGFVYTQPIAQWHNRGEQEVFEYCLEDGSIIRATKDHKFMTTDGQMLPIDEIFERGL

SEQ ID NO: 2 - protein, 101 aa, synthetic construct
  source 1..101: note = synthetic polypeptide
CLSYDTEILTVEYGFLPIGKIVEERIECTVYTVDKNGFVYTQPIAQWHNRGEQEVFEYCLEDGSIIRATKDHKFMTTDGQMLPIDEIFERGLDLKQVDGLP

SEQ ID NO: 3 - protein, 35 aa, synthetic construct
  source 1..35: note = synthetic polypeptide
VKIISRKSLGTQNVYDIGVEKDHNFLLKNGLVASN

SEQ ID NO: 4 - protein, 36 aa, synthetic construct
  source 1..36: note = synthetic polypeptide
MVKIISRKSLGTQNVYDIGVEKDHNFLLKNGLVASN

SEQ ID NO: 5 - protein, 102 aa, Nostoc punctiforme
CLSYETEILTVEYGLLPIGKIVEKRIECTVYSVDNNGNIYTQPVAQWHDRGEQEVFEYCLEDGSLIRATKDHKFMTVDGQMLPIDEIFERELDLMRVDNLPN

SEQ ID NO: 6 - protein, 35 aa, Nostoc punctiforme
IKIATRKYLGKQNVYDIGVERDHNFALKNGFIASN

SEQ ID NO: 7 - protein, 102 aa, Chroococcidiopsis thermalis
CLSYDTEILTVEYGAIPIGKIVEERIECTVYSVDNNGFIYTQPIAQWHNRGQQEVFEYCLEDGSIIRATKDHKFMTFEGKMLPIDEIFEQELDLKQVKSIQN

SEQ ID NO: 8 - protein, 35 aa, Chroococcidiopsis thermalis
VKIISRKSLGIQPVYDIGVERDHKFVLKNGLVASN

SEQ ID NO: 9 - protein, 102 aa, Nodularia spumigena
CLSYDTEILTVEYGYIPIGEIVEKAIECSVYSVDNNGNVYTQPIAQWHNRGEQEVFEYSLEDGSTIRATKDHKFMTTDGQMLPIDEIFAQELDLLQVHGLPK

SEQ ID NO: 10 - protein, 35 aa, Nodularia spumigena
VKITARKFVGRENVYDIGVERYHNFAIKNGLIASN

SEQ ID NO: 11 - protein, 102 aa, Anabaena cylindrica
CLSYDTEVLTVEYGFIPIGEIVEKRIECSIFSVDKNGNVYTQPIAQWHNRGRQEIYEYCLDDGSKIRATKDHKFMTTAGEMLPIDEIFERDLDLLKVEGLPE

SEQ ID NO: 12 - protein, 35 aa, Anabaena cylindrica
VKIISRQYLGQADVYDIGVEEDHNFAIKNGFIASN

SEQ ID NO: 13 - protein, 102 aa, Calothrix sp.
CLSYDTEVLTVEYGLLPIGEIVEKGIECRVFSVDNHGNVYTQPIAQWHNRGQQEVFEYGLDDGSVIRATKDHKFMTTDGKMLPIDEIFERGLDLLQVQGLPE

SEQ ID NO: 14 - protein, 35 aa, Calothrix sp.
VKVITRKYIGKENVYDIGVELDHNFAIRNGLVASN

SEQ ID NO: 15 - protein, 102 aa, Nostoc sp.
CLSYDTEILTVEYGFLPIGEIVEKGIECTVFSVASNGIVYTQPIAQWHNRGQQEIFEYCLEDGSIIRATKDHKFMTQDGQMLPIDEIFACELDLLQVQGLPE

SEQ ID NO: 16 - protein, 35 aa, Nostoc sp.
VKVVTRKYIGKENVYDIGVERDHNFVIRNGLVASN

SEQ ID NO: 17 - protein, 102 aa, Nostoc azollae
CLSYKTEVLTVEYGLIPIGEIVEKRIECSLFSVDENGNIYTQPIAQWHHRGVQEVYEYCLDDGTIIRATKDHKFMTTIGEMLPIDEIFERDLNLLQVNGLPT

SEQ ID NO: 18 - protein, 35 aa, Nostoc azollae
VKIISRQFLGPANVYDIGVAQDHNFAIKNGLIASN

SEQ ID NO: 19 - protein, 102 aa, Nostoc sp.
CLSYDTEVLTVEYGFVPIGEIVEKGIECSVFSINNNGIVYTQPIAQWHHRGKQEVFEYCLEDGSIIKATKDHKFMTQDGKMLPIDEIFEQELDLLQVKGLPE

SEQ ID NO: 20 - protein, 35 aa, Nostoc sp.
IKIASRKFLGVENVYDIGVRRDHNFFIKNGLIASN

SEQ ID NO: 21 - protein, 102 aa, Anabaena variabilis
CLSYDTEVLTVEYGFVPIGEIVDKGIECSVFSIDSNGIVYTQPIAQWHHRGKQEVFEYCLEDGSIIKATKDHKFMTQDGKMLPIDEIFEQELDLLQVKGLPE

SEQ ID NO: 22 - protein, 35 aa, Anabaena variabilis
IKIASRKFLGVENVYDIGVGRDHNFFVKNGLIASN

SEQ ID NO: 23 - protein, 100 aa, Pleurocapsa sp.
CLSYDTKILTVEYGAMPIGKIVEEQIDCTVYTVNQNGFVYTQPIAQWHDRGKQEIFEYCLEDGSIIRATKDHKFMTTDGQMLPIDKIFEKGLDLKTINCD

SEQ ID NO: 24 - protein, 35 aa, Pleurocapsa sp.
VKILSRKSLGIQSVYDIGVEKDHNFLLANGLVASN

SEQ ID NO: 25 - protein, 100 aa, Cyanothece sp.
CLSYETQIMTVEYGLMPIGKIVEEQIDCTVYTVNKNGFVYTQPIAQWHYRGEQEVFEYCLEDGSTIRATKDHKFMTTDGQMLPIDEIFEQGLELKQIHLS

SEQ ID NO: 26 - protein, 35 aa, Cyanothece sp.
VKIISRQSLGIQPVYDIGVEKDHNFLISDGLIASN

SEQ ID NO: 27 - protein, 99 aa, Cyanothece sp.
CLSYDTEILTVEYGPMPIGKIVEEQIECTVYTVDKNGLVYTQPIAQWHHRGQQEVFEYCLEDGSIIRATKDHKFMTDDGQMLPIEEIFEKGLELKQIIL

SEQ ID NO: 28 - protein, 35 aa, Cyanothece sp.
VKIISRQLAGNQTVYDLGVEKDHNFLLANGLIASN

SEQ ID NO: 29 - protein, 102 aa, Nostoc sp.
CLSYDTQVLTVEYGLVPIGEIVEKQLECSVFTIDGHGYVYTQAIAQWHNRGQQEVFEYGLEDGSVIRATKDHKFMTTDGQMLPIDEIFERELDLLQVQGLRW

SEQ ID NO: 30 - protein, 35 aa, Nostoc sp.
VKIITRKYIGQANVYDIGVAQDHNFVIENRLIASN

SEQ ID NO: 31 - protein, 101 aa, Tolypothrix bouteillei
CLSYDTEILTVEYGFLPIGKIVEKGIECNVYSVDKNGNIYTQPIAQWHDRGEQEVFEYCLENGSVIRATKDHKFMTTSGEMLPIDEIFERGLDLIRVEDLP

SEQ ID NO: 32 - protein, 35 aa, Tolypothrix bouteillei
VKILTRKSIGKQTVYDIGVERDHNFVIKNGSVASN

SEQ ID NO: 33 - protein, 101 aa, Aphanizomenon ovalisporum
  MOD_RES 87: note = X can be any amino acid
CLSADTEILTVEYGFLPIGEIVGKAIECRVYSVDGNGNIYTQSIAQWHNRGEQEVFEYTLEDGSIIRATKDHKFMTTDGEMLPIDEXFARQLDLMQVQGLH

SEQ ID NO: 34 - protein, 35 aa, Aphanizomenon ovalisporum
VKITARKFVGRENVYDIGVEHHHNFAIKNGLIASN

SEQ ID NO: 35 - protein, 102 aa, Oscillatoria nigro-viridis
CLSYDTKILTVEYGPMAIGKIVEEKIECTVYSVDSNGYIYTQSIAQWHRRGQQEVFEYCLEDGSIIRATKDHKFMTVGGQMLPIDEIFEQGLDLKQINSSSD

SEQ ID NO: 36 - protein, 35 aa, Oscillatoria nigro-viridis
VKIISRKSLGTQEVYDIGVEREHNFILENSLVASN

SEQ ID NO: 37 - protein, 100 aa, Rivularia sp.
CLSYDTEVLTEEFGLIPIGKIVEEKIDCTVYSVDVNGNVYSQPIAQWHNRGMQEVFEYELEDGSTIRATKDHKFMTVDGEMLAIDEIFEKGLELKRVGIY

SEQ ID NO: 38 - protein, 35 aa, Rivularia sp.
VKIISRKVLKTENVYDIGLEGDHNFIIKDGLIASN

SEQ ID NO: 39 - protein, 102 aa, Trichodesmium erythraeum
CLTYETEIMTVEYGPLPIGKIVEYRIECTVYTVDKNGYIYTQPIAQWHNRGMQEVYEYSLEDGTVIRATPEHKFMTEDGQMLPIDEIFERNLDLKCLGTLEL

SEQ ID NO: 40 - protein, 35 aa, Trichodesmium erythraeum
VKIVSRKLAKTENVYDIGVTKDHNFVLANGLIASN

SEQ ID NO: 41 - protein, 102 aa, Microcoleus sp.
CLSYDSEILTVEYGLMPIGKIVEEGIECTVYSVDSHGYLYTQPIAQWHHRGQQEVFEYDLEDGSVIRATKDHKFMTSEGQMLAIDEIFERGLELKQVKRSQP

SEQ ID NO: 42 - protein, 35 aa, Microcoleus sp.
VKIVRRKSLGIQTVYDIGVERDHNFLLANGLVASN

SEQ ID NO: 43 - protein, 102 aa, Stanieria cyanosphaera
CLSYDTEILTVEYGAMPIGKIVKEQIECNVYTVNQNGFIYPQAIAQWHERGKQEIFEYTLDNGLVIRATKDHKFMTIDGQMLPIDEIFERGLELQRINDYSN

SEQ ID NO: 44 - protein, 35 aa, Stanieria cyanosphaera
VKIVSRKSLGKQPVYDIGVTKDHNFLLSNGVVASN

SEQ ID NO: 45 - protein, 102 aa, Calothrix sp.
CLSYDTEILTWEYGFLKIGEIVEKQILCSVFSVDEQGNVYTQPIAQWHNRGLQELFAYQLEDGGVIRATKDHKFMTTDGQMLAIDEIFERQLDLFQVKGLPE

SEQ ID NO: 46 - protein, 35 aa, Calothrix sp.; identical to SEQ ID NO: 38

SEQ ID NO: 47 - protein, 99 aa, Cyanobacterium stanieri
CLSYDTEVLTVEYGVLPIGKIVEEQIQCTVYSVDQYGFVYTQAIAQWHDRGEQEVFEYELENGATIKATKDHKMMTSDGQMLPIDQIFEQGLDLFMVSF

SEQ ID NO: 48 - protein, 35 aa, Cyanobacterium stanieri
VKIVKRRSHGIQKVYDIGVAKDHNFLLHNGLVASN

SEQ ID NO: 49 - protein, 99 aa, Cyanothece sp.
CLSYDTEILTVEYGPMPIGKIVEENINCTVYTVDPNGFVYTQAIAQWHYRGEQEIFEYYLEDGATIRATKDHKFMTMEGKMLPIDEIFENNLDLKQLTL

SEQ ID NO: 50 - protein, 35 aa, Cyanothece sp.
VKIIGRQSLGVQKVYDIGVEKEHNFLLHNGLIASN

SEQ ID NO: 51 - protein, 99 aa, Cyanothece sp.
CLSYDTEILTVEYGAIPIGKVVEENIDCTVYTVDKNGFVYTQNIAQWHLRGQQEVFEYYLDDGSILRATKDHQFMTLEGEMLPIHEIFERGLELKKIKI

SEQ ID NO: 52 - protein, 35 aa, Cyanothece sp.
VKIVSYRSLGKQFVYDIGVAQDHNFLLANGSIASN

SEQ ID NO: 53 - protein, 101 aa, Anabaena sp.
CLSYDTEILTVEYGFLEIGEIVEKQIECKVYTIDSNGMLYTQSIAQWHNRGQQEVYEYLLENGAIIRATKDHKFMTEAGQMLPIDEIFAQGLDLLQVGVAE

SEQ ID NO: 54 - protein, 35 aa, Anabaena sp.
VKIVSRTYVGQANVYDIGVESDHNFVIKNGFIASN

SEQ ID NO: 55 - protein, 102 aa, Aphanothece halophytica
CLSYDTEIWTVEYGAMPIGKIVEEKIECSVYTVDENGFVYTQPIAQWHPRGQQEIIEYTLEDGRKIRATKDHKMMTESGEMLPIEEIFQRELDLKVETFHEM

SEQ ID NO: 56 - protein, 35 aa, Aphanothece halophytica
VKIIKRQSLGRQNVYDVCVETDHNFVLANGCVASN

SEQ ID NO: 57 - protein, 102 aa, Halothece sp.; identical to SEQ ID NO: 55

SEQ ID NO: 58 - protein, 35 aa, Halothece sp.
VKIIKRQSLGRQNVYDIGVETDHNFVLANGCVASN

SEQ ID NO: 59 - protein, 102 aa, Cyanobacterium aponinum
CLSYDTEILTVEYGAISIGKIVEEKINCQVYSVDKNGFIYTQNIAQWHDRGSQELFEYELEDGRIIKATKDHKMMTKDGQMLAINDIFEQELELYSVDDMGV

SEQ ID NO: 60 - protein, 35 aa, Cyanobacterium aponinum
VKIVKRRSLGVQPVYDIGVEKDHNFILANGLVASN

SEQ ID NO: 61 - protein, 98 aa, unidentified
  source 1..98: note = Candidatus Atelocyanobacterium thalassa isolate sequence
CLSYDTKVLTVEYGPLPIGKVVQENIRCRVYTTNDQGLIYTQPIAQWHNRGKQEIFEYHLDDKTIIRATKEHQFMTVDHVMMPIDEIFEQGLELKKIK

SEQ ID NO: 62 - protein, 35 aa, unidentified
  source 1..35: note = Candidatus Atelocyanobacterium thalassa isolate sequence
LKIIRRKSLGMHEVFDIGLEKDHNFVLSNGLIASN

SEQ ID NO: 63 - protein, 102 aa, Oscillatoria limnetica
CLSYNTEVLTVEYGPLPIGKIVDEQIHCRVYSVDENGFVYTQAIAQWHDRGYQEIFAYELADGSVIRATKDHQFMTEDGQMFPIDEIWEKGLDLKKLPTVQD

SEQ ID NO: 64 - protein, 35 aa, Oscillatoria limnetica
VKIVRRQSLGVQNVYDIGVEKDHNFLLASGEIASN

SEQ ID NO: 65 - protein, 102 aa, unidentified
  source 1..102: note = Cyanobacterium endosymbiont of Epithemia turgida sequence
CLSYDTEVLTVEYGAIPIGRMVEESLDCTVYTVDKNGFVYTQSIQQWHSRGQQEIFEYCFEDGSIIRATKDHKFMTAEGKMSSIHDIFEQGLELKKIIPWSG

SEQ ID NO: 66 - protein, 35 aa, unidentified
  source 1..35: note = Cyanobacterium endosymbiont of Epithemia turgida sequence
AKIISCKSLGKQSVYDIGVVQDHNFLLANGVVASN

SEQ ID NO: 67 - protein, 98 aa, Synechococcus sp.
CLGYDTPVLTVEYGFMPIGKIVEEKIQCHVYSVDQNGLVFTQAIAQWHNRGQQEVWEYNLDNGDIVRATKDHKFMTIDGQMLPINQIFEQGLELKVIA

SEQ ID NO: 68 - protein, 35 aa, Synechococcus sp.
VKIVSCKPLRVQTVYDIGVEKDHNFILDNGLVASN

SEQ ID NO: 69 - protein, 99 aa, Dactylococcopsis salina
CLSYDTEVLTEEYGAIPIGKIVEERMNCHVYSVDENGFIYSQPIAQWHPRGEQEVVEYTLEDGKIIRATADHKMMTETGEMLPIEQIFQQQLDLKISNQ

SEQ ID NO: 70 - protein, 35 aa, Dactylococcopsis salina
VKIINRQSLGKQTVYDIGVEKDHNFILGNGLVASN

SEQ ID NO: 71 - protein, 102 aa, Cylindrospermum stagnale
CLSYDTEILTVEYGFIPIGEIVEKRIECSVYSVDNHGNVYTQPIAQWHNRGLQEVFEYCLEDGSTIRATKDHKFMTTDKEMLPIDEIFERGLDLLRVEGLPI

SEQ ID NO: 72 - protein, 35 aa, Cylindrospermum stagnale
VKIIMRSYVGRENVYDIGVERDHNFVAKNGLIAAN

SEQ ID NO: 73 - protein, 102 aa, Synechocystis sp.
CLSFGTEILTVEYGPLPIGKIVSEEINCSVYSVDPEGRVYTQAIAQWHDRGEQEVLEYELEDGSVIRATSDHRFLTTDYQLLAIEEIFARQLDLLTLENIKQ

SEQ ID NO: 74 - protein, 35 aa, Synechocystis sp.
VKVIGRRSLGVQRIFDIGLPQDHNFLLANGAIAAN

SEQ ID NO: 75 - protein, 102 aa, Geitlerinema sp.
CLSYETPVMTVEYGPLPIGRIVEEQLDCTVYSVDEQGHVYTQPVAQWHHRGLQEVVEYELEDGRRLRATADHRFMTETGEMLPLAEIFERGLELRQVALRVP

SEQ ID NO: 76 - protein, 35 aa, Geitlerinema sp.
VKIVSRRSLGMQLVYDIGVAADHNFVLADGLIAAN

SEQ ID NO: 77 - protein, 102 aa, Synechocystis sp.
CLSFDAEILTVEYGPLSIGKIVGEEINCSVYSVDPQGRIYTQAIAQWHDRGVQEVFEYELEDGSVIRATPDHRFLTTDYELLAIEEIFARQMDLLTLTNLKL

SEQ ID NO: 78 - protein, 35 aa, Synechocystis sp.
VKVVRRRSLGMHRVFDIGLAQDHNFLLANGAIAAN

SEQ ID NO: 79 - protein, 100 aa, Microcystis aeruginosa
CLGGETLILTEEYGLLPIAKIVSEEVNCTVYSVDKNGFVYSQPISQWHERGLQEVFEYTLENGQTIQATKDHKFMTNDGEMLAIDTIFERGLDLKSSDFS

SEQ ID NO: 80 - protein, 35 aa, Microcystis aeruginosa
VKIISRQSLGRKPVYDIGVEKDHNFLLGNGLIASN

SEQ ID NO: 81 - protein, 100 aa, Microcystis aeruginosa
CLGGETLILTEEYGLLPIAKIVSEEINCTVYTVDQNGFVYSQPISQWHERGLQEVFEYTLENGQTIQATKDHKFMTSDGEMLAIDTIFERGLDLKSSDFS

SEQ ID NO: 82 - protein, 35 aa, Microcystis aeruginosa
VKIIGRQSLGRKPVYDIGVEKDHNFLLGNGLIASN

SEQ ID NO: 83 - protein, 102 aa, Acaryochloris marina
CLSYDTPVLTLEYGWLPIGQVVQEQIECQVFSINERGHLYTQPIAQWHHRGQQEVFEYTLADGSTIQATAEHQFMTTDGQMYPVQQIFEEGLSLKQLPLPWQ

SEQ ID NO: 84 - protein, 35 aa, Acaryochloris marina
VKIIQRRSLGLQSVYDIGLAQDHNFVMANGWVAAN

SEQ ID NO: 85 - protein, 102 aa, Leptolyngbya sp.
CLDGETPIVTVEYGVLPIREIVEKELLCSVYSIDENGFVYTQPVEQWHQRGDRQMFEYQLDNGGVIRATPDHKFLTTEGEMVAIDEIFEKGLNLAEFAPADL

SEQ ID NO: 86 - protein, 35 aa, Leptolyngbya sp.
VKILRRHSIGKAKTYDIGVSKNHNFLLANGLFASN

SEQ ID NO: 87 - protein, 102 aa, Synechococcus elongatus
CLAADTEVLTVEYGPIAIGKLVEENIRCQVYCCNPDGYIYSQPIGQWHQRGEQEVIEYELSDGRIIRATADHRFMTEEGEMLSLDEIFERSLELKQIPTPLL

SEQ ID NO: 88 - protein, 35 aa, Synechococcus elongatus
VKIVRRRSLGVQPVYDLGVATVHNFVLANGLVASN

SEQ ID NO: 89 - protein, 102 aa, Synechococcus sp.
CLSADTELYTVEYGWLPIGRLVEEQIECQVLSVNAHGHVYSQPIAQWHRRAWQEVFEYQLETGGTIKATTDHQFLTTDGQMYRIEDIFQRGLDLWQLPPDRF

SEQ ID NO: 90 - protein, 35 aa, Synechococcus sp.
VKIISRCSLGIQPVYDIGVAQDHNFVIRGGLVASN

SEQ ID NO: 91 - protein, 102 aa, Thermosynechococcus elongatus
CLSGETAVMTVEYGAVPIRRLVQERLSCHVYSLDGQGHLYTQPIAQWHFQGFRPVYEYQLEDGSTICATPDHRFMTTRGQMLPIEQIFQEGLELWQVAIAPR

SEQ ID NO: 92 - protein, 35 aa, Thermosynechococcus elongatus
GKIVGRRLMGWQAVYDIGLAADHNFVLANGAIAAN

SEQ ID NO: 93 - protein, 102 aa, Thermosynechococcus sp.
CLSGETAVMTVEYGAVPIRRLVQERLTCHVYSLDAQGHLYTQPIAQWHFQGFRPVYEYQLEDGSTIWATPDHRFMTTRGQMLPIEQIFQEGLELWQGPIAPS

SEQ ID NO: 94 - protein, 35 aa, Thermosynechococcus sp.
CKIVGRQLVGWQAVYDIGVARDHNFLLANGAIAAN

SEQ ID NO: 95 - protein, 102 aa, Thermosynechococcus vulcanus
CLSGETAVMTVEYGAIPIRRLVQERLICQVYSLDPQGHLYTQPIAQWHFQGFRPVYAYQLEDGSTICATPDHRFMTTSGQMLPIEQIFREGLELWQVAIAPP

SEQ ID NO: 96 - protein, 35 aa, Thermosynechococcus vulcanus
CKIVGRRLVGWQAVYDIGLAGDHNFLLANGAIAAN

SEQ ID NO: 97 - protein, 102 aa, Synechococcus sp.
CLAGGTPVVTVEYGVLPIQTIVEQELLCHVYSVDAQGLIYAQLIEQWHQRGDRLLYEYELENGQMIRATPDHRFLTTTGELLPIDEIFTQNLDLAAWAVPDS

SEQ ID NO: 98 - protein, 35 aa, Synechococcus sp.
VKIIRRKFIGHAPTYDIGLSQDHNFLLGQGLIAAN

SEQ ID NO: 99 - protein, 101 aa, Scytonema hofmanni
CLSYDTEVLTAEYGFLPIGKIVEKAIECTVYSVDNDGNIYTQPIAQWHDRGQQEVFEYSLDDGSVIRATKDHKFMTTGGQMLPIDEIFERGLDLMRIDSLP

SEQ ID NO: 100 - protein, 35 aa, Scytonema hofmanni
VKILTRKSIGKQTVYDIGVERDHNFVIKNGLVASN

SEQ ID NO: 101 - protein, 101 aa, Westiella intricata
CLSYDTEILTVEYGFLPIGEIVEKRIECTVYTVDTNGYVYTQAIAQWHNRGEQEVFEYALEDGSIIRATKDHKFMTSEGQMLPIDEIFVKGLDLLQVQGLP

SEQ ID NO: 102 - protein, 35 aa, Westiella intricata
VKIITRKFLGIQNVYDIGVEQNHNFVIKNGLVASN

SEQ ID NO: 103 - protein, 101 aa, Fischerella sp.
CLSYDTEILTVEYGFLPIGEIVEKGIECTVYTVDNNGNVYTQTIAQWHNRGQQEVFEYCLEDGSVIRATKDHKFMTTDGQMLPIDEIFARGLDLLQVKNLP

SEQ ID NO: 104 - protein, 35 aa, Fischerella sp.
VKIVTRRPLGTQNVYDIGVESDHNFVIKNGLVASN

SEQ ID NO: 105 - protein, 102 aa, Mastigocladopsis repens
CLSYDTEVLTVEYGFLPIGEIVEKSIECSVYTVDSNGNVYTQPIAQWHNRGQQEVFEYCLEDGSIIRATKDHKFMTIHGQMLPIDEIFERGLELMKIQGLPE

SEQ ID NO: 106 - protein, 35 aa, Mastigocladopsis repens
AKIITRKSLGTQNVYDIGVERDHNFVTRDGFIASN

SEQ ID NO: 107 - protein, 102 aa, Scytonema hofmanni
CLSYNSEVLTVEYGFLPIGKIVEKGIECSVYSVDSYGKIYTQVIAQWHNRGQQEVFEYCLEDGTIIQATKDHKFMTVDGQMLPIDEIFERGLDLMQVQGLPD

SEQ ID NO: 108 - protein, 35 aa, Scytonema hofmanni
VKIITRKSLGTQNVYDIGVSSDHNFVMKNGLIASN

SEQ ID NO: 109 - protein, 102 aa, Anabaena sp.
CLSSDTEVLTVEYGLIPIGEIIEKRIDCSVFSVDKNGNIYTQPIAQWHDRGIQELYEYCLDDGSTIRATKDHKFMTTAGEMLPIDEIFERGLDLLKVHNLPQ

SEQ ID NO: 110 - protein, 35 aa, Anabaena sp.
VKIITRNYVGKENVYDIGVERDHNFAIKNGLIASN

SEQ ID NO: 111 - protein, 102 aa, Fischerella sp.
CLSYDTEVLTVEYGFLPIGEIVEKRIECTVYTVDHNGYVYTQPIAQWHNRGYQEVFEYGLEDGSVIRATKDHKFMTSEGQMLPIDEIFARELDLLQVTGLVN

SEQ ID NO: 112 - protein, 35 aa, Fischerella sp.
VKIVTRRLLGIQNVYDIGVEQNHNFVIKNGLVASN

SEQ ID NO: 113 - protein, 102 aa, Calothrix sp.
CLSYDTEIFTVEYGFLPIGEIVEKRLECTVLTVDNHGNIYSQPIAQWHHRGQQQIYEYGLEDGSVIRATKDHKFMTTDGQMLPIDEIFERGLDLLQVTNLDN

SEQ ID NO: 114 - protein, 35 aa, Calothrix sp.
VKVITRKLADTENVYDIGVENHHNFLIKNGLVASN

SEQ ID NO: 115 - protein, 101 aa, Fischerella thermalis
CLSYETEILTVEYGFLPIGEIVEKRIECSVYTVDNNGYVCTQPIAQWHNRGYQEVFEYGLEDGSVIRATKDHKFMTIDRQMLPIDEIFARGLDLLQVTGLP

SEQ ID NO: 116 - protein, 35 aa, Fischerella thermalis
VKIITRKSLGTQNVYDIGVEQNHNFVIKNGLVASN

SEQ ID NO: 117 - protein, 102 aa, Cyanobacterium sp.
CLSYDTEILTVEYGFLSIGEIVEKEIECTVYTVDSNGYIYTQPIAQWHEQGEQEIFEYSLEDGSTIRATKDHKFMTIEGEMLPIDQIFARQLDLMQITGLPQ

SEQ ID NO: 118 - protein, 35 aa, Cyanobacterium sp.
VKISTKKSLGKQKVYDIGVVRDHNFIIKNGFVASN

SEQ ID NO: 119 - protein, 101 aa, Fischerella sp.
CLSYDTEVLTVEYGFLPIGEIVEKRIECTVYTVDTNGYVYTQAIAQWHNRDEQEVFEYALEDGSIIRATKDHKFMTSEGQMLPIDEIFAKGLDLLQVQGLP

SEQ ID NO: 120 - protein, 35 aa, Fischerella sp.
VKIVTRKFLGIQNVYDIGVEQNHNFVIKNGLVASN

SEQ ID NO: 121 - protein, 102 aa, Fischerella muscicola
CLSYETEILTVEYGFLPIGEIVEKRIECSVYTVDNNGYVCTQTIAQWHNRGYQEVFEYGLEDGSVIRATKDHKFMTIDRQMLPIDEIFARGLDLLQVKGLPE

SEQ ID NO: 122 - protein, 35 aa, Fischerella muscicola
VKIITRQSLGTQNVYDIGVEQNHNFVIKNGLVASN

SEQ ID NO: 123 - protein, 102 aa, Fischerella muscicola
CLSYDTEVLTVEYGFLPIGEIVEKTIECNVFTVDSNGYVYTQPIAQWHNRGYQEVFEYGLEDGSVIRATKDHKFMTSEGKMLPIDEIFARELDLLQVTGLIN

SEQ ID NO: 124 - protein, 35 aa, Fischerella muscicola; identical to SEQ ID NO: 120

SEQ ID NO: 125 - protein, 102 aa, Lyngbya aestuarii
CLSYDTEILTVEYGAIPIGKVVDEKIECTVYSVDKNGLIYTQPIAQWHNRGKQEVFEYSLEDGSTIRATKDHKFMTMDNQMLPIDEILEKGLELKQVNADSV

SEQ ID NO: 126 - protein, 35 aa, Lyngbya aestuarii
VKIVSRKSLDSQTVYDIGVETDHNFLLANGSVASN

SEQ ID NO: 127 - protein, 100 aa, Microchaete sp.
CLSYKTQVLTVEYGLLAIGEIVEKNIECSVFSVDIHGNVYTQPIAQWHHRGQQEVFEYGLEDGSIIRATKDHKFMTTQGEMLPIDEIFARGLDLLQVKGV

SEQ ID NO: 128 - protein, 35 aa, Microchaete sp.
VKIITRKYIGKENVYDIGVEQDHNFAIKNGLIAAN

SEQ ID NO: 129 - protein, 102 aa, Leptolyngbya sp.
CLSYDTEILTVEYGALPIGKIVENQMICSVYSIDNNGYIYIQPIAQWHNRGQQEVFEYILEDGSIIRSTKDHKFMTKGGEMLPIDEIFERGLELAQVTRLEQ

SEQ ID NO: 130 - protein, 35 aa, Leptolyngbya sp.
VKIISRRSVGVQSVYDIGVKQDHNFFLRNGLIASN

SEQ ID NO: 131 - protein, 102 aa, Crocosphaera watsonii
CLSYDTEILTVEYGAMYIGKIVEENINCTVYTVDKNGFVYTQTIAQWHNRGEQEIFEYDLEDGSKIKATKDHKFMTIDGEMLPIDEIFEKNLDLKQVVSHPD

SEQ ID NO: 132 - protein, 35 aa, Crocosphaera watsonii
VKIIGCRSLGTQKVYDIGVEKDHNFLLANGSIASN

SEQ ID NO: 133 - protein, 100 aa, Coleofasciculus chthonoplastes
CLSYDTQILTVEYGAVAIGEIVEKQIECTVYSVDENGYVYTQPIAQWHNRGEQEVFEYLLEDGATIRATKDHKFMTDEDQMLPIDQIFEQGLELKQVEVL

SEQ ID NO: 134 - protein, 35 aa, Coleofasciculus chthonoplastes
VKIIGRKPLGTQPVYDIGVERDHNFLLFNGSVASN

SEQ ID NO: 135 - protein, 98 aa, Chroococcidiopsis sp.
CLSYDTEVLTVEYGAIPIGKIVEEKIACNVYSVDKNGFVYTQPIAQYHDRGIQEVFEYRLENGSVIRATKDHKMMTADGQMLPIDEIFKQNLDLKQLN

SEQ ID NO: 136 - protein, 35 aa, Chroococcidiopsis sp.
VKIISRQSLGKQSVFDIGVAKDHNFLLANGLVASN

SEQ ID NO: 137 - protein, 97 aa, Aphanizomenon flos-aquae
CLSYDTEILTVEYGFLQIGEIVEKQIECKVYTVDSNGILYTQSIAQWHNRGQQEVYEYLLENGAIIRATKDHKFMTEEGQMLPIDEIFSQGLDLLQV

SEQ ID NO: 138 - protein, 35 aa, Aphanizomenon flos-aquae
VKIISRTYVGQANVYDIGVENDHNFVIKNGFIAAN

SEQ ID NO: 139 - protein, 102 aa, Raphidiopsis brookii
CLSYETEVLTLEYGFLPIGEIVDKQMVCTVFSVNDSGNVYTQPIGQWHDRGVQELYEYCLDDGSTIRATKDHKFMTTQGEMVPIDEIFHQGWELVQVSGTMN

SEQ ID NO: 140 - protein, 35 aa, Raphidiopsis brookii
VKIVSRRYLGKADVYDIGVAKDHNFIIKNGLVASN

SEQ ID NO: 141 - protein, 99 aa, Cyanothece sp.
CLSYDTEILTVEYGPMPIGKIVEENINCSVYTVNKNGFVYTQSIAQWHHRGEQEVFEYYLEDGETIRATKDHKFMTTEGKMLPIDEIFENNLDLKKLTV

SEQ ID NO: 142 - protein, 35 aa, Cyanothece sp.
VKIIERRSLGKQNVYDIGVEKDHNFLLSNNLIASN

SEQ ID NO: 143 - protein, 100 aa, Xenococcus sp.
CLSADTEVLTVEYGAISIGKIVEERIECTVYSVDANGFVYTQEIAQWHNRGEQEVFEYMLDDGSVIRATKDHKLMTIDGQMVAIDEIFSQGLELKQVLGL

SEQ ID NO: 144 - protein, 35 aa, Xenococcus sp.
VKIVSRKSLGTQTVYDLGVARDHNFLLANGTVASN

SEQ ID NO: 145 - protein, 100 aa, Pleurocapsa sp.
CLSYDTEIYTVEYGALPIGKIVESRIKCTVLTVDKNGLVYSQPIVQWHDRGIQEVFEYTLDNGATIRATKDHKFMTVEGQMLPIDEIFELGLELKEIQQF

SEQ ID NO: 146 - protein, 35 aa, Pleurocapsa sp.
VKIISRQSLGKQSVYDIGVAKDHNFLLANGMVASN

SEQ ID NO: 147 - protein, 102 aa, Cylindrospermopsis raciborskii
CLSYETEVLTLEYGFVPIGEIVNKQMVCTVFSLNDSGNVYTQPIGQWHDRGVQDLYEYCLDDGSTIRATKDHKFMTTQGEMVPIDEIFHQGWELVQVSGISK

SEQ ID NO: 148 - protein, 35 aa, Cylindrospermopsis raciborskii; identical to SEQ ID NO: 140

SEQ ID NO: 149 - protein, 94 aa, Spirulina major
CLTYDTLVLTVEYGPVPIGKLVEAQINCQVYSVDANGFIYTQAIAQWHDRGQRQVYEYTLEDGSTIRATPDHKFMTATGEMLPIDQIFEQGLDL

SEQ ID NO: 150 - protein, 35 aa, Spirulina major
VKIIHRRALPPQSVYDIGVERDHNFLLPSGWVASN

SEQ ID NO: 151 - protein, 96 aa, Spirulina subsalsa
CLSYDTKIITVEYGAIAIGTIVEQGLHCHVYSVDPNGFIYTQPIAQWHQRGEQEVFAYTLENGSIIQATKDHKFMTQQGKMLPIDTIFEQGLDLLQ

SEQ ID NO: 152 - protein, 35 aa, Spirulina subsalsa
VKIIKRTSLGVRPVYDIGVIQDHNFLLENGLVASN

SEQ ID NO: 153 - protein, 100 aa, Microcystis aeruginosa
CLGGETLILTEEYGLLPIAKIVSEEINCTVYSVDKNGFIYSQPISQWHERGLQEVFEYTLENGQTIQATKDHKFMTSDGEMLAIDTIFERGLDLKSSDFS

SEQ ID NO: 154 - protein, 35 aa, Microcystis aeruginosa
VKIISRQFLGRKPVYDIGVEKDHNFLLGNGLIASN

SEQ ID NO: 155 - protein, 95 aa, Myxosarcina sp.
CLSYDTEVLTLKYGALPIGEIVEKRINCHVYTRAESGFFYIQSIEQWHDRGEQEVFEYTLENGATIKATKDHKFMTSGGQMLPIDEIFERGLDLL

SEQ ID NO: 156 - protein, 35 aa, Myxosarcina sp.
VKIVSRKSLGKQPVYDLGVAKDHNFLLANGTVASN

SEQ ID NO: 157 - protein, 101 aa, Leptolyngbya sp.
CLSADTQLLTVEYGPLEIGRIVEEQIACHVYSVDANGFVYTQPIAQWHSRGEQEIFEYQLEDGRTLRATADHKFMTTTGEMGRINDIFEQGLDLKQIDLPQ

SEQ ID NO: 158 - protein, 35 aa, Leptolyngbya sp.
VKVVSRQSLGVQPVYDIGVATDHNFLLADGLVASN

SEQ ID NO: 159 - protein, 97 aa, Acaryochloris sp.
CLSYDTPVLTLEYGWLPIGQVVQEQIECQVFSINERGHLYTQPIAQWHHRGQQEVFEYTLTDGSTIQATAEHQFMTTDGQMYPIQQIFEEGLSLKQL

SEQ ID NO: 160 - protein, 35 aa, Acaryochloris sp.
VKITQRRSLGLQSVYDIGLAQDHNFVIANGWVAAN

SEQ ID NO: 161 - protein, 98 aa, Geminocystis herdmanii
CLSYDTEVLTVEFGAIPMGKIVEERLNCQVYSVDKNGFIYTQNIAQWHDRGVQEVFEYELEDGRIIKATKDHKMMIENCEMVEIDRIFEEGLELFEVN

SEQ ID NO: 162 - protein, 35 aa, Geminocystis herdmanii
VKILKRRSISSQQVYDIGVEKDHNFLLANGLVASN

SEQ ID NO: 163 - protein, 98 aa, Nodosilinea nodulosa
CLSADTELLTLEYGPLTIGEIVAKRIPCHVFSVDESGYVYTQPVAQWHQRGHQEVFEYQLDDGTTIRATADHQFMTELGEMMAIDEIFQRGLELKQVE

SEQ ID NO: 164 - protein, 35 aa, Nodosilinea nodulosa
VKIISRQSLGVQPVYDIGVARDHNFLLADGQVASN

SEQ ID NO: 165 - protein, 102 aa, Rubidibacter lacunae
CLSYDTEVLTVEYGPLAIGTIVSERLACTVYTVDRSGFLYAQAISQWHERGRQDVFEYALDNGMTIRATKDHKLMTADGQMVAIDDIFTQGLTLKAIDTAAF

SEQ ID NO: 166 - protein, 35 aa, Rubidibacter lacunae
MKIVSRKSLGVQHVYDIGVARDHNFLLANGAIASN

SEQ ID NO: 167 - protein, 101 aa, Chlorogloeopsis fritschii
CLSYDTAILTVEYGFLPIGEIVEKGIECTVYTVDSNGYIYTQPIAQWHNRGEQELFEYSLEDGSIIRATKDHKFMTIDGQMLPIDEIFARKLELMQVKGLP

SEQ ID NO: 168 - protein, 35 aa, Chlorogloeopsis fritschii
VKIIAKKSLGTQNVYDIGVERDHNFVIKNGLVASN

SEQ ID NO: 169 - protein, 102 aa, Richelia intracellularis
CLSYDTQILTVEHGPMSIGEIVEKCLECHVYTVNKNGNICIQTITQWHFRGEQEIFEYELEDGSFIQATKDHKFMTTTGEMLPIHEIFTNGLEILQLSKSLL

SEQ ID NO: 170 - protein, 35 aa, Richelia intracellularis
VKILARKSLGTQKVYDIGVNDDHNFALSNSFIASN

SEQ ID NO: 171 - protein, 102 aa, Synechococcus sp.
CLAGDTPVVTVEYGVLPIQTIVEQELLCQVYSVDAQGLIYTQPIEQWHNRGDRLLYEYELENGQMIRATPDHKFLTTTGELLPIDEIFTQNLDLAAWAVPDS

SEQ ID NO: 172 - protein, 35 aa, Synechococcus sp.; identical to SEQ ID NO: 98

SEQ ID NO: 173 - protein, 102 aa, Synechococcus sp.
CLAGDTPVVTVEYGVLPIQTIVEQELLCHVYSVDAQGLIYTQPIEQWHQRGDRFLYEYELENGQMIRATPDHKFLTTTGKLLPIDEIFTQNLDLAAWAVPDS

SEQ ID NO: 174 - protein, 35 aa, Synechococcus sp.
VKIIRRKFIGHAPTYDIGLSQDHNFLLGQGFIAAN

SEQ ID NO: 175 - protein, 102 aa, Synechococcus sp.
CLAGDTPVVTVEYGVLPIQTIVEQELLCHVYSVDAQGLIYTQPIEQWHQRGDRLLYEYELENGQMIRATPDHKFLTTTGELLPIDEIFTQNLDLAAWAVPDS

SEQ ID NO: 176 - protein, 35 aa, Synechococcus sp.
VKILRRKFIGRAPTYDIGLSQDHNFLLGQGLVAAN

SEQ ID NO: 177 - protein, 94 aa, Synechococcus sp.
CLAGDTPVVTVEYGVLPIRTIVDQELLCHVYSLDPQGFIYAQPVEQWHRRGDRLLYEYELETGAVIRATPDHKFLTATGEMLPIDEIFVRNLDL

SEQ ID NO: 178 - protein, 35 aa, Synechococcus sp.
VKIIRRNLIGEAATYDIGLGKDHNFLLGQGLIASN

SEQ ID NO: 179 - protein, 95 aa, Synechococcus sp.
CLAGGTPVVTVEYGVLPIQTIVEQELLCHVYSVDAQGLIYTQPIEQWHQRGDRLLYEYELENGQMIRATPDHKFLTTTGELLPIDEIFTQNLDLL

SEQ ID NO: 180 - protein, 35 aa, Synechococcus sp.; identical to SEQ ID NO: 98

SEQ ID NO: 181 - protein, 95 aa, Synechococcus sp.
CLAGDTPVVTVEYGVLPIQTIVEQELLCHVYSVDAQGLIYTQPIEQWHKRGDRLLYEYELENGQIIRATPDHKFLTTTGEMRPIDEIFAKNLSLL

SEQ ID NO: 182 - protein, 35 aa, Synechococcus sp.
VKIIRRKFVGHAPTYDIGLSQDHNFLLGQGLIAAN

SEQ ID NO: 183 - protein, 99 aa, Cyanothece sp.; identical to SEQ ID NO: 51

SEQ ID NO: 184 - protein, 35 aa, Cyanothece sp.; identical to SEQ ID NO: 52

SEQ ID NO: 185 - protein, 102 aa, Synechococcus elongatus; identical to SEQ ID NO: 87

SEQ ID NO: 186 - protein, 35 aa, Synechococcus elongatus; identical to SEQ ID NO: 88

SEQ ID NO: 187 - protein, 102 aa, Chlorogloeopsis fritschii
CLSYDTAILTVEYGFLPIGEIVEKGIECTVYTVDSNGYIYTQPIAQWHNRGEQELFEYSLEDGSIIRATKDHKFMTIDGQMLPIDEIFARKLELMQVKGLPE

SEQ ID NO: 188 - protein, 35 aa, Chlorogloeopsis fritschii; identical to SEQ ID NO: 168

SEQ ID NO: 189 - protein, 97 aa, Cyanothece sp.
CLSYDTEILTVEYGPMPIGKIVEENINCTVYTVDPNGFVYTQAIAQWHYRGEQEIFEYYLEDGATIRATKDHKFMTMEGKMLPIDEIFENNLDLKQL

SEQ ID NO: 190 - protein, 35 aa, Cyanothece sp.; identical to SEQ ID NO: 50

SEQ ID NO: 191 - protein, 97 aa, Lyngbya majuscula
CLSYDTEIITVEYGPIAIGEIVEKGIPCTVYSVDSNGYVYTQPIAQWHNRGEQEVFEYTLDDGSVIRATKDHKFMTIDGQMLPIDEIFEGGLELKQL

SEQ ID NO: 192 - protein, 35 aa, Lyngbya majuscula
VKIISRKSLGTQPVYDIGVKDDHNFILANGMVASN

SEQ ID NO: 193 - protein, 102 aa, unidentified
  source 1..102: note = filamentous cyanobacterium ESFC-1 sequence
CLSYDTEVLTVEYGAVPIGKLVEEKLNCSVYTVDPNGYIYTQAIAQWHDRGIQEVFEYQLEDNTIIRATKDHKFMTEDHQMLPIDEIFERGLELKKCPQPQQ

SEQ ID NO: 194 - protein, 35 aa, unidentified
  source 1..35: note = filamentous cyanobacterium ESFC-1 sequence
VKIIRRRSLGFQPVYDIGLEQDHNFLLNQGAIASN

SEQ ID NO: 195 - protein, 94 aa, Synechococcus sp.
CLAGGTPVVTVEYGVLPIQTIVEQELLCHVYSVDAQGLIYAQLIEQWHQRGDRLLYEYELENGQMIRATPDHRFLTTTGELLPIDEIFTQNLDL

SEQ ID NO: 196 - protein, 35 aa, Synechococcus sp.; identical to SEQ ID NO: 98

SEQ ID NO: 197 - protein, 97 aa, Acaryochloris marina
CLSYDTPVLTLEYGWLPIGQVVQEQIECQVFSINERGHLYTQPIAQWHHRGQQEVFEYTLADGSTIQATAEHQFMTTDGQMYPVQQIFEEGLSLKQL

SEQ ID NO: 198 - protein, 35 aa, Acaryochloris marina; identical to SEQ ID NO: 84

SEQ ID NO: 199 - protein, 94 aa, Microcystis aeruginosa
CLGGETLILTEEYGLLPIAKIVSEEVNCTVYSVDKNGFVYSQPISQWHERGLQEVFEYTLENGQTIQATKDHKFMTNDGEMLAIDTIFERGLDL

SEQ ID NO: 200 - protein, 35 aa, Microcystis aeruginosa; identical to SEQ ID NO: 80

SEQ ID NO: 201 - protein, 90 aa, Anabaena circinalis
CLSYDTEILTVEYGFLEIGEIVEKQIECKVYTVDSNGILYTQPIAQWHHRGQQEVYEYLLENGAIIRATKDHKFMTEAGEMLPIDDIFTQ

SEQ ID NO: 202 - protein, 35 aa, Anabaena circinalis
VKIISRTYVGQANVYDIGVENDHNFVIKNGFVAAN

SEQ ID NO: 203 - protein, 90 aa, Anabaena circinalis
CLSYDTEILTVEYGFLEIGEIVEKQIECRVYTVDSNGILYTQPIAQWHYRGQQEVYEYLLENGAIIRATKDHNFMTEAGEMLPIDDIFTQ

SEQ ID NO: 204 - protein, 35 aa, Anabaena circinalis
IKIISRKYVGQANVYDIGVENDHNFVIKNGFVAAN

SEQ ID NO: 205 - protein, 90 aa, Cyanobacterium sp.
CLSYDTKVLTVEYGPLPIGKVVQENIRCRVYTTNDQGLIYTQPIAQWHNRGKQEIFEYHLDDKTIIRATKEHQFMTVDHVMMPIDEIFEQ

SEQ ID NO: 206 - protein, 34 aa, Cyanobacterium sp.
KIIRRKSLGMHEVFDIGLEKDHNFVLSNGLIASN

SEQ ID NO: 207 - protein, 94 aa, Planktothrix sp.
CLSYDTEVLTVEYGLIPISKIVEEKIECTVYTVNNQGYVYTQPIAQWHNRGEQEVFEYYLEDGSVIRATKDHKFMTVEGQMLPIDEIFEKELDL

SEQ ID NO: 208 - protein, 35 aa, Planktothrix sp.
VKIISRKSLGTQPVYDIGVQEDHNFVLNNGLVASN

SEQ ID NO: 209 - protein, 94 aa, Planktothrix sp.
CLSYDTEILTVEYGLMPIGKIVKEKIECTVYTVNNQGYVYTQPIAQWHHRGEQEVFEYCLEDGSVIRATKDHKFMTVQGQMLPIDEIFEKELDL

SEQ ID NO: 210 - protein, 35 aa, Planktothrix sp.
VKIISRKSLGTQPVYDIGVQEDHNFLLNNGLVASN

SEQ ID NO: 211 - protein, 102 aa, Fremyella diplosiphon
CLSYDTEVLTVEYGLIPIGEIVEKRLECSVYSVDINGNVYTQPIAQWHHRGQQEVFEYALEDGSIIRATKDHKFMTTDGQMLPIDEIFERGLDLLQVPHLPE

SEQ ID NO: 212 - protein, 35 aa, Fremyella diplosiphon
VKIVTRRAIGAANVYDIGVEQDHNFAIKNGLIAAN

SEQ ID NO: 213 - protein, 94 aa, Planktothrix sp.
CLSYDTEILTVEYGLIPISKIVEEKIECTVYTVNNQGYVYTQPIAQWHNRGEQEVFEYYLEDGSVIRATKDHKFMTVDGQMLPIDEIFEKELDL

SEQ ID NO: 214 - protein, 35 aa, Planktothrix sp.; identical to SEQ ID NO: 208

SEQ ID NO: 215 - protein, 102 aa, Nostoc punctiforme; identical to SEQ ID NO: 5

SEQ ID NO: 216 - protein, 35 aa, Nostoc punctiforme; identical to SEQ ID NO: 6

SEQ ID NO: 217 - protein, 102 aa, Chroococcidiopsis thermalis; identical to SEQ ID NO: 7

SEQ ID NO: 218 - protein, 35 aa, Chroococcidiopsis thermalis; identical to SEQ ID NO: 8

SEQ ID NO: 219 - protein, 102 aa, Nodularia spumigena; identical to SEQ ID NO: 9

SEQ ID NO: 220 - protein, 35 aa, Nodularia spumigena; identical to SEQ ID NO: 10

SEQ ID NO: 221 - protein, 102 aa, Anabaena cylindrica; identical to SEQ ID NO: 11

SEQ ID NO: 222 - protein, 35 aa, Anabaena cylindrica; identical to SEQ ID NO: 12

SEQ ID NO: 223 - protein, 102 aa, Calothrix sp.; identical to SEQ ID NO: 13

SEQ ID NO: 224 - protein, 35 aa, Calothrix sp.; identical to SEQ ID NO: 14

SEQ ID NO: 225 - protein, 102 aa, Nostoc sp.; identical to SEQ ID NO: 15

SEQ ID NO: 226 - protein, 35 aa, Nostoc sp.; identical to SEQ ID NO: 16

SEQ ID NO: 227 - protein, 102 aa, Nostoc azollae; identical to SEQ ID NO: 17

SEQ ID NO: 228 - protein, 35 aa, Nostoc azollae; identical to SEQ ID NO: 18

SEQ ID NO: 229 - protein, 102 aa, Nostoc sp.; identical to SEQ ID NO: 19

SEQ ID NO: 230 - protein, 35 aa, Nostoc sp.; identical to SEQ ID NO: 20

SEQ ID NO: 231 - protein, 102 aa, Anabaena variabilis; identical to SEQ ID NO: 21

SEQ ID NO: 232 - protein, 35 aa, Anabaena variabilis; identical to SEQ ID NO: 22

SEQ ID NO: 233 - protein, 100 aa, Pleurocapsa sp.; identical to SEQ ID NO: 23

SEQ ID NO: 234 - protein, 35 aa, Pleurocapsa sp.; identical to SEQ ID NO: 24

SEQ ID NO: 235 - protein, 100 aa, Cyanothece sp.; identical to SEQ ID NO: 25

SEQ ID NO: 236 - protein, 35 aa, Cyanothece sp.; identical to SEQ ID NO: 26

SEQ ID NO: 237 - protein, 99 aa, Cyanothece sp.; identical to SEQ ID NO: 27

SEQ ID NO: 238 - protein, 35 aa, Cyanothece sp.; identical to SEQ ID NO: 28

SEQ ID NO: 239 - protein, 102 aa, Nostoc sp.; identical to SEQ ID NO: 29

SEQ ID NO: 240 - protein, 35 aa, Nostoc sp.; identical to SEQ ID NO: 30

SEQ ID NO: 241 - protein, 101 aa, Tolypothrix bouteillei; identical to SEQ ID NO: 31

SEQ ID NO: 242 - protein, 35 aa, Tolypothrix bouteillei; identical to SEQ ID NO: 32

SEQ ID NO: 243 - protein, 101 aa, Aphanizomenon ovalisporum; identical to SEQ ID NO: 33
  MOD_RES 87: note = Any amino acid

SEQ ID NO: 244 - protein, 35 aa, Aphanizomenon ovalisporum; identical to SEQ ID NO: 34

SEQ ID NO: 245 - protein, 102 aa, Oscillatoria nigro-viridis; identical to SEQ ID NO: 35

SEQ ID NO: 246 - protein, 35 aa, Oscillatoria nigro-viridis; identical to SEQ ID NO: 36

SEQ ID NO: 247 - protein, 100 aa, Rivularia sp.; identical to SEQ ID NO: 37

SEQ ID NO: 248 - protein, 35 aa, Rivularia sp.; identical to SEQ ID NO: 38

SEQ ID NO: 249 - protein, 102 aa, Microcoleus sp.; identical to SEQ ID NO: 41

SEQ ID NO: 250 - protein, 35 aa, Microcoleus sp.; identical to SEQ ID NO: 42

SEQ ID NO: 251 - protein, 102 aa, Stanieria cyanosphaera; identical to SEQ ID NO: 43

SEQ ID NO: 252 - protein, 35 aa, Stanieria cyanosphaera; identical to SEQ ID NO: 44

SEQ ID NO: 253 - protein, 102 aa, Calothrix sp.; identical to SEQ ID NO: 45

SEQ ID NO: 254 - protein, 35 aa, Calothrix sp.; identical to SEQ ID NO: 38

SEQ ID NO: 255 - protein, 99 aa, Cyanobacterium stanieri; identical to SEQ ID NO: 47

SEQ ID NO: 256 - protein, 35 aa, Cyanobacterium stanieri; identical to SEQ ID NO: 48

SEQ ID NO: 257 - protein, 99 aa, Cyanothece sp.; identical to SEQ ID NO: 49

SEQ ID NO: 258 - protein, 35 aa, Cyanothece sp.; identical to SEQ ID NO: 50

SEQ ID NO: 259 - protein, 99 aa, Cyanothece sp.; identical to SEQ ID NO: 51

SEQ ID NO: 260 - protein, 35 aa, Cyanothece sp.; identical to SEQ ID NO: 52

SEQ ID NO: 261 - protein, 101 aa, Anabaena sp.; identical to SEQ ID NO: 53

SEQ ID NO: 262 - protein, 35 aa, Anabaena sp.; identical to SEQ ID NO: 54

SEQ ID NO: 263 - protein, 102 aa, Aphanothece halophytica; identical to SEQ ID NO: 55

SEQ ID NO: 264 - protein, 35 aa, Aphanothece halophytica; identical to SEQ ID NO: 56

SEQ ID NO: 265 - protein, 102 aa, Halothece sp.; identical to SEQ ID NO: 55

SEQ ID NO: 266 - protein, 35 aa, Halothece sp.; identical to SEQ ID NO: 58

SEQ ID NO: 267 - protein, 102 aa, Cyanobacterium aponinum; identical to SEQ ID NO: 59

SEQ ID NO: 268 - protein, 35 aa, Cyanobacterium aponinum; identical to SEQ ID NO: 60

SEQ ID NO: 269 - protein, 98 aa, unidentified; identical to SEQ ID NO: 61
  source 1..98: note = Candidatus Atelocyanobacterium thalassa isolate sequence

SEQ ID NO: 270 - protein, 35 aa, unidentified; identical to SEQ ID NO: 62
  source 1..35: note = Candidatus Atelocyanobacterium thalassa isolate sequence

SEQ ID NO: 271 - protein, 102 aa, Oscillatoria limnetica; identical to SEQ ID NO: 63

SEQ ID NO: 272 - protein, 35 aa, Oscillatoria limnetica; identical to SEQ ID NO: 64

SEQ ID NO: 273 - protein, 102 aa, unidentified; identical to SEQ ID NO: 65
  source 1..102: note = Cyanobacterium endosymbiont of Epithemia turgida sequence

SEQ ID NO: 274 - protein, 35 aa, unidentified; identical to SEQ ID NO: 66
  source 1..35: note = Cyanobacterium endosymbiont of Epithemia turgida sequence

SEQ ID NO: 275 - protein, 98 aa, Synechococcus sp.; identical to SEQ ID NO: 67

SEQ ID NO: 276 - protein, 35 aa, Synechococcus sp.; identical to SEQ ID NO: 68

SEQ ID NO: 277 - protein, 90 aa, Cyanobacterium sp.; identical to SEQ ID NO: 205

SEQ ID NO: 278 - protein, 34 aa, Cyanobacterium sp.; identical to SEQ ID NO: 206

SEQ ID NO: 279 - protein, 94 aa, Planktothrix sp.; identical to SEQ ID NO: 207

SEQ ID NO: 280 - protein, 35 aa, Planktothrix sp.; identical to SEQ ID NO: 208

SEQ ID NO: 281 - protein, 94 aa, Planktothrix sp.; identical to SEQ ID NO: 209

SEQ ID NO: 282 - protein, 35 aa, Planktothrix sp.; identical to SEQ ID NO: 210

SEQ ID NO: 283 - protein, 94 aa, Planktothrix sp.; identical to SEQ ID NO: 213

SEQ ID NO: 284 - protein, 35 aa, Planktothrix sp.; identical to SEQ ID NO: 208

SEQ ID NO: 285 - protein, 99 aa, Cyanothece sp.; identical to SEQ ID NO: 51

SEQ ID NO: 286 - protein, 35 aa, Cyanothece sp.; identical to SEQ ID NO: 52

SEQ ID NO: 287 - protein, 102 aa, Chlorogloeposis fritschii; identical to SEQ ID NO: 187

SEQ ID NO: 288 - protein, 35 aa, Chlorogloeposis fritschii; identical to SEQ ID NO: 168

SEQ ID NO: 289 - protein, 97 aa, Cyanothece sp.; identical to SEQ ID NO: 189

SEQ ID NO: 290 - protein, 35 aa, Cyanothece sp.; identical to SEQ ID NO: 50

SEQ ID NO: 291 - protein, 97 aa, Lyngbya majuscula; identical to SEQ ID NO: 191

SEQ ID NO: 292 - protein, 35 aa, Lyngbya majuscula; identical to SEQ ID NO: 192

SEQ ID NO: 293 - protein, 102 aa, unidentified; identical to SEQ ID NO: 193
  source 1..102: note = filamentous cyanobacterium ESFC-1 sequence

SEQ ID NO: 294 - protein, 35 aa, unidentified; identical to SEQ ID NO: 194
  source 1..35: note = filamentous cyanobacterium ESFC-1 sequence

SEQ ID NO: 295 - protein, 94 aa, Microcystis aeruginosa; identical to SEQ ID NO: 199

SEQ ID NO: 296 - protein, 35 aa, Microcystis aeruginosa; identical to SEQ ID NO: 80

SEQ ID NO: 297 - protein, 102 aa, Rubidibacter lacunae; identical to SEQ ID NO: 165

SEQ ID NO: 298 - protein, 35 aa, Rubidibacter lacunae; identical to SEQ ID NO: 166

SEQ ID NO: 299 - protein, 101 aa, Chlorogloeopsis fritschii; identical to SEQ ID NO: 167

SEQ ID NO: 300 - protein, 35 aa, Chlorogloeopsis fritschii; identical to SEQ ID NO: 168

SEQ ID NO: 301 - protein, 102 aa, Richelia intracellularis; identical to SEQ ID NO: 169

SEQ ID NO: 302 - protein, 35 aa, Richelia intracellularis; identical to SEQ ID NO: 170

SEQ ID NO: 303 - protein, 98 aa, Geminocystis herdmanii; identical to SEQ ID NO: 161

SEQ ID NO: 304 - protein, 35 aa, Geminocystis herdmanii; identical to SEQ ID NO: 162

SEQ ID NO: 305 - protein, 97 aa, Spirulina subsalsa
CLSYDTKIITVEYGAIAIGTIVEQGLHCHVYSVDPNGFIYTQPIAQWHQRGEQEVFAYTLENGSIIQATKDHKFMTQQGKMLPIDTIFEQGLDLLQV

SEQ ID NO: 306 - protein, 34 aa, Spirulina subsalsa
KIIKRTSLGVRPVYDIGVIQDHNFLLENGLVASN

SEQ ID NO: 307 - protein, 100 aa, Microcystis aeruginosa; identical to SEQ ID NO: 153

SEQ ID NO: 308 - protein, 35 aa, Microcystis aeruginosa; identical to SEQ ID NO: 154

SEQ ID NO: 309 - protein, 95 aa, Myxosarcina sp.; identical to SEQ ID NO: 155

SEQ ID NO: 310 - protein, 35 aa, Myxosarcina sp.; identical to SEQ ID NO: 156

SEQ ID NO: 311 - protein, 101 aa, Scytonema hofmanni; identical to SEQ ID NO: 99

SEQ ID NO: 312 - protein, 35 aa, Scytonema hofmanni; identical to SEQ ID NO: 100

SEQ ID NO: 313 - protein, 101 aa, Westiella intricata; identical to SEQ ID NO: 101

SEQ ID NO: 314 - protein, 35 aa, Westiella intricata; identical to SEQ ID NO: 102

SEQ ID NO: 315 - protein, 101 aa, Fischerella sp.; identical to SEQ ID NO: 103

SEQ ID NO: 316 - protein, 35 aa, Fischerella sp.; identical to SEQ ID NO: 104

SEQ ID NO: 317 - protein, 102 aa, Mastigocladopsis repens; identical to SEQ ID NO: 105

SEQ ID NO: 318 - protein, 35 aa, Mastigocladopsis repens; identical to SEQ ID NO: 106

SEQ ID NO: 319 - protein, 102 aa, Scytonema hofmanni; identical to SEQ ID NO: 107

SEQ ID NO: 320 - protein, 35 aa, Scytonema hofmanni; identical to SEQ ID NO: 108

SEQ ID NO: 321 - protein, 102 aa, Anabaena sp.; identical to SEQ ID NO: 109

SEQ ID NO: 322 - protein, 35 aa, Anabaena sp.; identical to SEQ ID NO: 110

SEQ ID NO: 323 - protein, 102 aa, Fischerella sp.; identical to SEQ ID NO: 111

SEQ ID NO: 324 - protein, 35 aa, Fischerella sp.; identical to SEQ ID NO: 112

SEQ ID NO: 325 - protein, 102 aa, Calothrix sp.; identical to SEQ ID NO: 113

SEQ ID NO: 326 - protein, 35 aa, Calothrix sp.; identical to SEQ ID NO: 114

SEQ ID NO: 327 - protein, 101 aa, Fischerella thermalis; identical to SEQ ID NO: 115

SEQ ID NO: 328 - protein, 35 aa, Fischerella thermalis; identical to SEQ ID NO: 116

SEQ ID NO: 329 - protein, 102 aa, unidentified; identical to SEQ ID NO: 117
  source 1..102: note = cyanobacterium PCC 7702 Chl7702 sequence

SEQ ID NO: 330 - protein, 35 aa, unidentified; identical to SEQ ID NO: 118
  source 1..35: note = cyanobacterium PCC 7702 Chl7702 sequence

SEQ ID NO: 331 - protein, 101 aa, Fischerella sp.; identical to SEQ ID NO: 119

SEQ ID NO: 332 - protein, 35 aa, Fischerella sp.; identical to SEQ ID NO: 120

SEQ ID NO: 333 - protein, 102 aa, Fischerella muscicola; identical to SEQ ID NO: 121

SEQ ID NO: 334 - protein, 35 aa, Fischerella muscicola; identical to SEQ ID NO: 122

SEQ ID NO: 335 - protein, 102 aa, Fischerella muscicola; identical to SEQ ID NO: 123

SEQ ID NO: 336 - protein, 35 aa, Fischerella muscicola; identical to SEQ ID NO: 120

SEQ ID NO: 337 - protein, 102 aa, Lyngbya aestuarii; identical to SEQ ID NO: 125

SEQ ID NO: 338 - protein, 35 aa, Lyngbya aestuarii; identical to SEQ ID NO: 126

SEQ ID NO: 339 - protein, 102 aa, Leptolyngbya sp.; identical to SEQ ID NO: 129

SEQ ID NO: 340 - protein, 35 aa, Leptolyngbya sp.; identical to SEQ ID NO: 130

SEQ ID NO: 341 - protein, 102 aa, Crocosphaera watsonii; identical to SEQ ID NO: 131

SEQ ID NO: 342 - protein, 35 aa, Crocosphaera watsonii; identical to SEQ ID NO: 132

SEQ ID NO: 343 - protein, 100 aa, Coleofasciculus chthonoplastes; identical to SEQ ID NO: 133

SEQ ID NO: 344 - protein, 35 aa, Coleofasciculus chthonoplastes; identical to SEQ ID NO: 134

SEQ ID NO: 345 - protein, 98 aa, Chroococcidiopsis sp.; identical to SEQ ID NO: 135

SEQ ID NO: 346 - protein, 35 aa, Chroococcidiopsis sp.; identical to SEQ ID NO: 136

SEQ ID NO: 347 - protein, 102 aa, Raphidiopsis brookii; identical to SEQ ID NO: 139

SEQ ID NO: 348 - protein, 35 aa, Raphidiopsis brookii; identical to SEQ ID NO: 140

SEQ ID NO: 349 - protein, 99 aa, Cyanothece sp.; identical to SEQ ID NO: 141

SEQ ID NO: 350 - protein, 35 aa, Cyanothece sp.; identical to SEQ ID NO: 142

SEQ ID NO: 351 - protein, 100 aa, Xenococcus sp.; identical to SEQ ID NO: 143

SEQ ID NO: 352 - protein, 35 aa, Xenococcus sp.; identical to SEQ ID NO: 144

SEQ ID NO: 353 - protein, 100 aa, Pleurocapsa sp.; identical to SEQ ID NO: 145

SEQ ID NO: 354 - protein, 35 aa, Pleurocapsa sp.; identical to SEQ ID NO: 146

SEQ ID NO: 355 - protein, 102 aa, Cylindrospermopsis raciborskii; identical to SEQ ID NO: 147

SEQ ID NO: 356 - protein, 35 aa, Cylindrospermopsis raciborskii; identical to SEQ ID NO: 140

SEQ ID NO: 357 - protein, 100 aa, Microcystis aeruginosa; identical to SEQ ID NO: 79

SEQ ID NO: 358 - protein, 35 aa, Microcystis aeruginosa; identical to SEQ ID NO: 80

SEQ ID NO: 359 - protein, 100 aa, Microcystis aeruginosa; identical to SEQ ID NO: 81

SEQ ID NO: 360 - protein, 35 aa, Microcystis aeruginosa; identical to SEQ ID NO: 82

SEQ ID NO: 361 - protein, 245 aa, synthetic construct
  source 1..245: note = synthetic polypeptide
MGSSHHHHHHGSGLVPRGSASMSDSEVNQEAKPEVKPEVKPETHINLKVSDGSSEIFFKIKKTTPLRRLMEAFAKRQGKEMDSLRFLYDGIRIQADQTPEDLDMEDNDIIEAHREQIGGAEYCLSFGTEILTVEYGPLPIGKIVSEEINCSVYSVDPEGRVYTQAIAQWHDRGEQEVLEYELEDGSVIRATSDHRFLTTDYQLLAIEEIFARQLDLLTLENIKQTEEALDNHRLPFPLLDAGTIK

SEQ ID NO: 362 - protein, 224 aa, synthetic construct
  source 1..224: note = synthetic polypeptide
MGSSHHHHHHGSGLVPRGSASMSDSEVNQEAKPEVKPEVKPETHINLKVSDGSSEIFFKIKKTTPLRRLMEAFAKRQGKEMDSLRFLYDGIRIQADQTPEDLDMEDNDIIEAHREQIGGAEYALSYETEILTVEYGLLPIGKIVEKRIECTVYSVDNNGNIYTQPVAQWHDRGEQEVFEYCLEDGSLIRATKDHKFMTVDGQMLPIDEIFERELDLMRVDNLPN

SEQ ID NO: 363 - protein, 240 aa, synthetic construct
  source 1..240: note = synthetic polypeptide
MVKVIGRRSLGVQRIFDIGLPQDHNFLLANGAIAANCITGDALVALPEGESVRIADIVPGARPNSDNAIDLKVLDRHGNPVLADRLFHSGEHPVYTVRTVEGLRVTGTANHPLLCLVDVAGVPTLLWKLIDEIKPGDYAVIQRSAFSVDCAGFARGKPEFAPTTYTVGVPGLVRFLEAHHRDPDAQAIADELTDGRFYYAKVASVTDAGVQPVYSLRVDTADHAFITNGFVSHAHHHHHH

SEQ ID NO: 364 - protein, 240 aa, synthetic construct
  source 1..240: note = synthetic polypeptide
MIKIATRKYLGKQNVYDIGVERDHNFALKNGFIASNCITGDALVALPEGESVRIADIVPGARPNSDNAIDLKVLDRHGNPVLADRLFHSGEHPVYTVRTVEGLRVTGTANHPLLCLVDVAGVPTLLWKLIDEIKPGDYAVIQRSAFSVDCAGFARGKPEFAPTTYTVGVPGLVRFLEAHHRDPDAQAIADELTDGRFYYAKVASVTDAGVQPVYSLRVDTADHAFITNGFVSHAHHHHHH

SEQ ID NO: 365 - protein, 245 aa, synthetic construct
  source 1..245: note = synthetic polypeptide
MGSSHHHHHHGSGLVPRGSASMSDSEVNQEAKPEVKPEVKPETHINLKVSDGSSEIFFKIKKTTPLRRLMEAFAKRQGKEMDSLRFLYDGIRIQADQTPEDLDMEDNDIIEAHREQIGGAEYCLSFGTEILTVEYGPLPIGKIVSEEINCSVYSVDPEGRVYTQAIAQWHDRGEQEVLEYELEDGSVIRATSDHKFMTTDGQMLAIEEIFARQLDLLTLENIKQTEEALDNHRLPFPLLDAGTIK

SEQ ID NO: 366 - protein, 245 aa, synthetic construct
  source 1..245: note = synthetic polypeptide
MGSSHHHHHHGSGLVPRGSASMSDSEVNQEAKPEVKPEVKPETHINLKVSDGSSEIFFKIKKTTPLRRLMEAFAKRQGKEMDSLRFLYDGIRIQADQTPEDLDMEDNDIIEAHREQIGGAEYCLSFGTEILTVEYGPLPIGKIVSEEINCSVYSVDPEGRVYTQAIAQWHDRGEQEVLEYELEDGSVIRATSDHKFLTTDYQLLAIEEIFARQLDLLTLENIKQTEEALDNHRLPFPLLDAGTIK

SEQ ID NO: 367 - protein, 245 aa, synthetic construct
  source 1..245: note = synthetic polypeptide
MGSSHHHHHHGSGLVPRGSASMSDSEVNQEAKPEVKPEVKPETHINLKVSDGSSEIFFKIKKTTPLRRLMEAFAKRQGKEMDSLRFLYDGIRIQADQTPEDLDMEDNDIIEAHREQIGGAEYCLSFGTEILTVEYGPLPIGKIVSEEINCSVYSVDPEGRVYTQAIAQWHDRGEQEVLEYELEDGSVIRATSDHKFLTTDGQLLAIEEIFARQLDLLTLENIKQTEEALDNHRLPFPLLDAGTIK

SEQ ID NO: 368 - protein, 245 aa, synthetic construct
  source 1..245: note = synthetic polypeptide
MGSSHHHHHHGSGLVPRGSASMSDSEVNQEAKPEVKPEVKPETHINLKVSDGSSEIFFKIKKTTPLRRLMEAFAKRQGKEMDSLRFLYDGIRIQADQTPEDLDMEDNDIIEAHREQIGGAEYCLSFGTEILTVEYGPLPIGKIVSEEINCSVYSVDPEGRVYTQAIAQWHDRGEQEVLEYELEDGSVIRATSDHKFLTTDGQMLAIEEIFARQLDLLTLENIKQTEEALDNHRLPFPLLDAGTIK

SEQ ID NO: 369 - protein, 245 aa, synthetic construct
  source 1..245: note = synthetic polypeptide
MGSSHHHHHHGSGLVPRGSASMSDSEVNQEAKPEVKPEVKPETHINLKVSDGSSEIFFKIKKTTPLRRLMEAFAKRQGKEMDSLRFLYDGIRIQADQTPEDLDMEDNDIIEAHREQIGGAEYCLSFGTEILTVEYGPLPIGKIVSEEINCSVYSVDPEGRVYTQAIAQWHDRGEQEVFEYELEDGSVIRATKDHRFLTTDYQLLPIDEIFARQLDLLTLENIKQTEEALDNHRLPFPLLDAGTIK

SEQ ID NO: 370 - protein, 245 aa, synthetic construct
  source 1..245: note = synthetic polypeptide
MGSSHHHHHHGSGLVPRGSASMSDSEVNQEAKPEVKPEVKPETHINLKVSDGSSEIFFKIKKTTPLRRLMEAFAKRQGKEMDSLRFLYDGIRIQADQTPEDLDMEDNDIIEAHREQIGGAEYCLSFGTEILTVEYGPLPIGKIVSEEINCSVYSVDPEGRVYTQAIAQWHDRGEQEVLEYELEDGSVIRATSDHRFLTTDYQLLPIEEIFARQLDLLTLENIKQTEEALDNHRLPFPLLDAGTIK

SEQ ID NO: 371 - protein, 245 aa, synthetic construct
  source 1..245: note = synthetic polypeptide
MGSSHHHHHHGSGLVPRGSASMSDSEVNQEAKPEVKPEVKPETHINLKVSDGSSEIFFKIKKTTPLRRLMEAFAKRQGKEMDSLRFLYDGIRIQADQTPEDLDMEDNDIIEAHREQIGGAEYCLSFGTEILTVEYGPLPIGKIVSEEINCSVYSVDPEGRVYTQAIAQWHDRGEQEVLEYELEDGSVIRATKDHRFLTTDYQLLPIEEIFARQLDLLTLENIKQTEEALDNHRLPFPLLDAGTIK

SEQ ID NO: 372 - protein, 245 aa, synthetic construct
  source 1..245: note = synthetic polypeptide
MGSSHHHHHHGSGLVPRGSASMSDSEVNQEAKPEVKPEVKPETHINLKVSDGSSEIFFKIKKTTPLRRLMEAFAKRQGKEMDSLRFLYDGIRIQADQTPEDLDMEDNDIIEAHREQIGGAEYCLSFGTEILTVEYGPLPIGKIVSEEINCSVYSVDPEGRVYTQAIAQWHDRGEQEVFEYELEDGSVIRATKDHRFLTTDYQLLPIEEIFARQLDLLTLENIKQTEEALDNHRLPFPLLDAGTIK

SEQ ID NO: 373 - protein, 245 aa, synthetic construct
  source 1..245: note = synthetic polypeptide
MGSSHHHHHHGSGLVPRGSASMSDSEVNQEAKPEVKPEVKPETHINLKVSDGSSEIFFKIKKTTPLRRLMEAFAKRQGKEMDSLRFLYDGIRIQADQTPEDLDMEDNDIIEAHREQIGGAEYCLSFGTEILTVEYGPLPIGKIVEKRIECSVYSVDPEGRVYTQAIAQWHDRGEQEVLEYELEDGSVIRATSDHRFLTTDYQLLAIEEIFARQLDLLTLENIKQTEEALDNHRLPFPLLDAGTIK

SEQ ID NO: 374 - protein, 245 aa, synthetic construct
  source 1..245: note = synthetic polypeptide
MGSSHHHHHHGSGLVPRGSASMSDSEVNQEAKPEVKPEVKPETHINLKVSDGSSEIFFKIKKTTPLRRLMEAFAKRQGKEMDSLRFLYDGIRIQADQTPEDLDMEDNDIIEAHREQIGGAEYCLSFGTEILTVEYGPLPIGKIVSEEINCSVYSVDNNGNIYTQAIAQWHDRGEQEVLEYELEDGSVIRATSDHRFLTTDYQLLAIEEIFARQLDLLTLENIKQTEEALDNHRLPFPLLDAGTIK

SEQ ID NO: 375 - protein, 240 aa, synthetic construct
  source 1..240: note = synthetic polypeptide
MIKIATRRSLGVQRIFDIGLPQDHNFLLANGAIAANCITGDALVALPEGESVRIADIVPGARPNSDNAIDLKVLDRHGNPVLADRLFHSGEHPVYTVRTVEGLRVTGTANHPLLCLVDVAGVPTLLWKLIDEIKPGDYAVIQRSAFSVDCAGFARGKPEFAPTTYTVGVPGLVRFLEAHHRDPDAQAIADELTDGRFYYAKVASVTDAGVQPVYSLRVDTADHAFITNGFVSHAHHHHHH

SEQ ID NO: 376 - protein, 240 aa, synthetic construct
  source 1..240: note = synthetic polypeptide
MVKVIGRRSLGVQNVYDIGLPQDHNFLLANGAIAANCITGDALVALPEGESVRIADIVPGARPNSDNAIDLKVLDRHGNPVLADRLFHSGEHPVYTVRTVEGLRVTGTANHPLLCLVDVAGVPTLLWKLIDEIKPGDYAVIQRSAFSVDCAGFARGKPEFAPTTYTVGVPGLVRFLEAHHRDPDAQAIADELTDGRFYYAKVASVTDAGVQPVYSLRVDTADHAFITNGFVSHAHHHHHH

SEQ ID NO: 377 - protein, 240 aa, synthetic construct
  source 1..240: note = synthetic polypeptide
MVKVIGRRSLGVQRIFDIGVERDHNFLLANGAIAANCITGDALVALPEGESVRIADIVPGARPNSDNAIDLKVLDRHGNPVLADRLFHSGEHPVYTVRTVEGLRVTGTANHPLLCLVDVAGVPTLLWKLIDEIKPGDYAVIQRSAFSVDCAGFARGKPEFAPTTYTVGVPGLVRFLEAHHRDPDAQAIADELTDGRFYYAKVASVTDAGVQPVYSLRVDTADHAFITNGFVSHAHHHHHH

SEQ ID NO: 378 - protein, 240 aa, synthetic construct
  source 1..240: note = synthetic polypeptide
MVKVIGRRSLGVQRIFDIGLPQDHNFALKNGFIAANCITGDALVALPEGESVRIADIVPGARPNSDNAIDLKVLDRHGNPVLADRLFHSGEHPVYTVRTVEGLRVTGTANHPLLCLVDVAGVPTLLWKLIDEIKPGDYAVIQRSAFSVDCAGFARGKPEFAPTTYTVGVPGLVRFLEAHHRDPDAQAIADELTDGRFYYAKVASVTDAGVQPVYSLRVDTADHAFITNGFVSHAHHHHHH

SEQ ID NO: 379 - protein, 240 aa, synthetic construct
  source 1..240: note = synthetic polypeptide
MVKVIGRRSLGVQRIFDIGLPQDHNFLLANGAIASNCITGDALVALPEGESVRIADIVPGARPNSDNAIDLKVLDRHGNPVLADRLFHSGEHPVYTVRTVEGLRVTGTANHPLLCLVDVAGVPTLLWKLIDEIKPGDYAVIQRSAFSVDCAGFARGKPEFAPTTYTVGVPGLVRFLEAHHRDPDAQAIADELTDGRFYYAKVASVTDAGVQPVYSLRVDTADHAFITNGFVSHAHHHHHH

SEQ ID NO: 380 - protein, 411 aa, synthetic construct
  source 1..411: note = synthetic polypeptide
TGCCTGTCTTACGACACAGAGATTCTGACCGTTGAATATGGATTCCTTCCTATCGGTAAGATCGTGGAGGAACGGATTGAATGCACAGTCTATACGGTAGATAAAAATGGCTTTGTGTATACACAACCTATTGCTCAGTGGCATAACCGGGGAGAACAGGAAGTTTTCGAATACTGCTTAGAAGACGGTTCGATTATCCGTGCAACGAAAGATCACAAATTTATGACGACCGACGGTCAGATGTTACCGATTGATGAGATTTTCGAACGGGGGTTAGACCTGAAACAAGTTGATGGTTTGCCGATGGTCAAGATCATTAGTCGTAAGAGTCTGGGCACTCAAAACGTCTACGATATTGGAGTAGAAAAAGATCATAATTTTTTGCTGAAGAATGGGCTGGTGGCCTCTAAC

SEQ ID NO: 381 - protein, 223 aa, synthetic construct
  source 1..223: note = synthetic polypeptide
MGSSHHHHHHGSGLVPRGSASMSDSEVNQEAKPEVKPEVKPETHINLKVSDGSSEIFFKIKKTTPLRRLMEAFAKRQGKEMDSLRFLYDGIRIQADQTPEDLDMEDNDIIEAHREQIGGAEYCLSYDTEILTVEYGFLPIGKIVEERIECTVYTVDKNGFVYTQPIAQWHNRGEQEVFEYCLEDGSIIRATKDHKFMTTDGQMLPIDEIFERGLDLKQVDGLP

SEQ ID NO: 382 - protein, 240 aa, synthetic construct
  source 1..240: note = synthetic polypeptide
MVKIISRKSLGTQNVYDIGVEKDHNFLLKNGLVASNCITGDALVALPEGESVRIADIVPGARPNSDNAIDLKVLDRHGNPVLADRLFHSGEHPVYTVRTVEGLRVTGTANHPLLCLVDVAGVPTLLWKLIDEIKPGDYAVIQRSAFSVDCAGFARGKPEFAPTTYTVGVPGLVRFLEAHHRDPDAQAIADELTDGRFYYAKVASVTDAGVQPVYSLRVDTADHAFITNGFVSHAHHHHHH

SEQ ID NO: 383 - skipped

SEQ ID NO: 384 - protein, 299 aa, synthetic construct
  source 1..299: note = synthetic polypeptide
MEQKLISEEDLSHIQRETSCSRPRLNSNMDADLYGYKWARDNVGQSGATIYRLYGKPDAPELFLKHGKGSVANDVTDEMVRLNWLTEFMPLPTIKHFIRTPDDAWLLTTAIPGKTAFQVLEEYPDSGENIVDALAVFLRRLHSIPVCNCPFNSDRVFRLAQAQSRMNNGLVDASDFDDERNGWPVEQVWKEMHKLLPFCLSYDTEILTVEYGFLPIGKIVEERIECTVYTVDKNGFVYTQPIAQWHNRGEQEVFEYCLEDGSIIRATKDHKFMTTDGQMLPIDEIFERGLDLKQVDGLP

SEQ ID NO: 385 - protein, 119 aa, synthetic construct
  MOD_RES 38: note = X can be F, G, R or E
  source 1..119: note = synthetic polypeptide
MVKIISRKSLGTQNVYDIGVEKDHNFLLKNGLVASNCXNSVVTHGDFSLDNLIFDEGKLIGCIDVGRVGIADRYQDLAILWNCLGEFSPSLQKRLFQKYGIDNPDMNKLQFHLMLDEFF

SEQ ID NO: 386 - protein, 408 aa, synthetic construct
  source 1..408: note = synthetic polypeptide
TGCCTGAGCTACGACACCGAGATCCTGACCGTGGAGTACGGCTTCCTGCCCATCGGCAAGATCGTGGAGGAGCGCATCGAGTGCACCGTGTACACCGTGGACAAGAACGGCTTCGTGTACACCCAGCCCATCGCCCAGTGGCACAACCGCGGCGAGCAGGAGGTGTTCGAGTACTGCCTGGAGGACGGCAGCATCATCCGCGCCACCAAGGACCACAAGTTCATGACCACCGACGGCCAGATGCTGCCCATCGACGAGATCTTCGAGCGCGGCCTGGACCTGAAGCAGGTGGACGGCCTGCCCGTGAAGATCATCAGCCGCAAGAGCCTGGGCACCCAGAACGTGTACGACATCGGCGTGGAGAAGGACCACAACTTCCTGCTGAAGAACGGCCTGGTGGCCAGCAAC

SEQ ID NO: 387 - protein, 580 aa, synthetic construct
  source 1..580: note = synthetic polypeptide
MGWSCIILFLVATATGVHSEVKLLESGGGLVQPGGSLRLSCAASGFTFNDFYMNWIRQPPGQAPEWLGVIRNKGNGYTTEVNTSVKGRFTISRDNTQNILYLQMNSLRAEDTAIYYCARGGPYYYSGDDAPYWGQGVMVTVSSATTKGPSVYPLAPGSAAQTNSMVTLGCLVKGYFPEPVTVTWNSGSLSSGVHTFPAVLQSDLYTLSSSVTVPSSTWPSETVTCNVAHPASSTKVDKKIVPRDCGCKPCICTVPEVSSVFIFPPKPKDVLTITLTPKVTCVVVAISKDDPEVQFSWFVDDVEVHTAQTQPREEQFNSTFRSVSELPIMHQDWLNGKEFKCRVNSAAFPAPIEKTISKTKGRPKAPQVYTIPPPKEQMAKDKVSLTCMITDFFPEDITVEWQWNGQPAENYKNTQPIMDTDGSYFVYSKLNVQKSNWEAGNTFTCSVLHEGLHNHHTEKSLSHSPGKASGGCLSYDTEILTVEYGFLPIGKIVEERIECTVYTVDKNGFVYTQPIAQWHNRGEQEVFEYCLEDGSIIRATKDHKFMTTDGQMLPIDEIFERGLDLKQVDGLPGHHHHHHG

SEQ ID NO: 388 - protein, 255 aa, synthetic construct
  source 1..255: note = synthetic polypeptide
MGHHHHHHSGVKIISRKSLGTQNVYDIGVEKDHNFLLKNGLVASNCFNSGGCITGDALVALPEGESVRIADIVPGARPNSDNAIDLKVLDRHGNPVLADRLFHSGEHPVYTVRTVEGLRVTGTANHPLLCLVDVAGVPTLLWKLIDEIKPGDYAVIQRSAFSVDCAGFARGKPEFAPTTYTVGVPGLVRFLEAHHRDPDAQAIADELTDGRFYYAKVASVTDAGVQPVYSLRVDTADHAFITNGFVSHAHHHHHH

SEQ ID NO: 389 - protein, 35 aa, synthetic construct
  source 1..35: note = synthetic polypeptide
VKIISRKSLGTQNVYDIGVGEPHNFLLKNGLVASN

SEQ ID NO: 390 - protein, 136 aa, synthetic construct
  source 1..136: note = synthetic polypeptide
CLSYDTEILTVEYGFLPIGKIVEERIECTVYTVDKNGFVYTQPIAQWHNRGEQEVFEYCLEDGSIIRATKDHKFMTTDGQMLPIDEIFERGLDLKQVDGLPVKIISRKSLGTQNVYDIGVEKDHNFLLKNGLVASN

SEQ ID NO: 391 - protein, 136 aa, synthetic construct
  source 1..136: note = synthetic polypeptide
CLSYDTEILTVEYGFLPIGKIVEERIECTVYTVDKNGFVYTQPIAQWHNRGEQEVFEYCLEDGSIIRATKDHKFMTTDGQMLPIDEIFERGLDLKQVDGLPVKIISRKSLGTQNVYDIGVGEPHNFLLKNGLVASN

SEQ ID NO: 392 - protein, 137 aa, synthetic construct
  source 1..137: note = synthetic polypeptide
CLSYETEILTVEYGLLPIGKIVEKRIECTVYSVDNNGNIYTQPVAQWHDRGEQEVFEYCLEDGSLIRATKDHKFMTVDGQMLPIDEIFERELDLMRVDNLPNIKIATRKYLGKQNVYDIGVERDHNFALKNGFIASN

SEQ ID NO: 393 - protein, 136 aa, synthetic construct
  source 1..136: note = synthetic polypeptide
CLSYDTEILTVEYGFLPIGKIVEERIECNTYSTDKNGFVYTQPIAQWHNRGEQEVFEYCLEDGSIIRATKDHKFMTTDGQMLPIDEIFERGLDLKQVDGLPVKIISRKSLGTQNVYDIGVEKDHNFLLKNGLVASN

SEQ ID NO: 394 - protein, 137 aa, Nostoc punctiforme; identical to SEQ ID NO: 392

SEQ ID NO: 395 - protein, 137 aa, Chroococcidiopsis thermalis
CLSYDTEILTVEYGAIPIGKIVEERIECTVYSVDNNGFIYTQPIAQWHNRGQQEVFEYCLEDGSIIRATKDHKFMTFEGKMLPIDEIFEQELDLKQVKSIQNVKIISRKSLGIQPVYDIGVERDHKFVLKNGLVASN

SEQ ID NO: 396 - protein, 137 aa, Nodularia spumigena
CLSYDTEILTVEYGYIPIGEIVEKAIECSVYSVDNNGNVYTQPIAQWHNRGEQEVFEYSLEDGSTIRATKDHKFMTTDGQMLPIDEIFAQELDLLQVHGLPKVKITARKFVGRENVYDIGVERYHNFAIKNGLIASN

SEQ ID NO: 397 - protein, 137 aa, Anabaena cylindrica
CLSYDTEVLTVEYGFIPIGEIVEKRIECSIFSVDKNGNVYTQPIAQWHNRGRQEIYEYCLDDGSKIRATKDHKFMTTAGEMLPIDEIFERDLDLLKVEGLPEVKIISRQYLGQADVYDIGVEEDHNFAIKNGFIASN

SEQ ID NO: 398 - protein, 137 aa, Calothrix sp.
CLSYDTEVLTVEYGLLPIGEIVEKGIECRVFSVDNHGNVYTQPIAQWHNRGQQEVFEYGLDDGSVIRATKDHKFMTTDGKMLPIDEIFERGLDLLQVQGLPEVKVITRKYIGKENVYDIGVELDHNFAIRNGLVASN

SEQ ID NO: 399 - protein, 137 aa, Nostoc sp.
CLSYDTEILTVEYGFLPIGEIVEKGIECTVFSVASNGIVYTQPIAQWHNRGQQEIFEYCLEDGSIIRATKDHKFMTQDGQMLPIDEIFACELDLLQVQGLPEVKVVTRKYIGKENVYDIGVERDHNFVIRNGLVASN

SEQ ID NO: 400 - protein, 137 aa, Nostoc azollae
CLSYKTEVLTVEYGLIPIGEIVEKRIECSLFSVDENGNIYTQPIAQWHHRGVQEVYEYCLDDGTIIRATKDHKFMTTIGEMLPIDEIFERDLNLLQVNGLPTVKIISRQFLGPANVYDIGVAQDHNFAIKNGLIASN

SEQ ID NO: 401 - protein, 137 aa, Nostoc sp.
CLSYDTEVLTVEYGFVPIGEIVEKGIECSVFSINNNGIVYTQPIAQWHHRGKQEVFEYCLEDGSIIKATKDHKFMTQDGKMLPIDEIFEQELDLLQVKGLPEIKIASRKFLGVENVYDIGVRRDHNFFIKNGLIASN

SEQ ID NO: 402 - protein, 137 aa, Anabaena variabilis
CLSYDTEVLTVEYGFVPIGEIVDKGIECSVFSIDSNGIVYTQPIAQWHHRGKQEVFEYCLEDGSIIKATKDHKFMTQDGKMLPIDEIFEQELDLLQVKGLPEIKIASRKFLGVENVYDIGVGRDHNFFVKNGLIASN

SEQ ID NO: 403 - protein, 135 aa, Pleurocapsa sp.
CLSYDTKILTVEYGAMPIGKIVEEQIDCTVYTVNQNGFVYTQPIAQWHDRGKQEIFEYCLEDGSIIRATKDHKFMTTDGQMLPIDKIFEKGLDLKTINCDVKILSRKSLGIQSVYDIGVEKDHNFLLANGLVASN

SEQ ID NO: 404 - protein, 135 aa, Cyanothece sp.
CLSYETQIMTVEYGLMPIGKIVEEQIDCTVYTVNKNGFVYTQPIAQWHYRGEQEVFEYCLEDGSTIRATKDHKFMTTDGQMLPIDEIFEQGLELKQIHLSVKIISRQSLGIQPVYDIGVEKDHNFLISDGLIASN

SEQ ID NO: 405 - protein, 134 aa, Cyanothece sp.
CLSYDTEILTVEYGPMPIGKIVEEQIECTVYTVDKNGLVYTQPIAQWHHRGQQEVFEYCLEDGSIIRATKDHKFMTDDGQMLPIEEIFEKGLELKQIILVKIISRQLAGNQTVYDLGVEKDHNFLLANGLIASN

SEQ ID NO: 406 - protein, 137 aa, Nostoc sp.
CLSYDTQVLTVEYGLVPIGEIVEKQLECSVFTIDGHGYVYTQAIAQWHNRGQQEVFEYGLEDGSVIRATKDHKFMTTDGQMLPIDEIFERELDLLQVQGLRWVKIITRKYIGQANVYDIGVAQDHNFVIENRLIASN

SEQ ID NO: 407 - protein, 136 aa, Tolypothrix bouteillei
CLSYDTEILTVEYGFLPIGKIVEKGIECNVYSVDKNGNIYTQPIAQWHDRGEQEVFEYCLENGSVIRATKDHKFMTTSGEMLPIDEIFERGLDLIRVEDLPVKILTRKSIGKQTVYDIGVERDHNFVIKNGSVASN

SEQ ID NO: 408 - protein, 136 aa, Aphanizomenon ovalisporum
  MOD_RES 87: note = Any amino acid
CLSADTEILTVEYGFLPIGEIVGKAIECRVYSVDGNGNIYTQSIAQWHNRGEQEVFEYTLEDGSIIRATKDHKFMTTDGEMLPIDEXFARQLDLMQVQGLHVKITARKFVGRENVYDIGVEHHHNFAIKNGLIASN

SEQ ID NO: 409 - protein, 137 aa, Oscillatoria nigro-viridis
CLSYDTKILTVEYGPMAIGKIVEEKIECTVYSVDSNGYIYTQSIAQWHRRGQQEVFEYCLEDGSIIRATKDHKFMTVGGQMLPIDEIFEQGLDLKQINSSSDVKIISRKSLGTQEVYDIGVEREHNFILENSLVASN

SEQ ID NO: 410 - protein, 135 aa, Rivularia sp.
CLSYDTEVLTEEFGLIPIGKIVEEKIDCTVYSVDVNGNVYSQPIAQWHNRGMQEVFEYELEDGSTIRATKDHKFMTVDGEMLAIDEIFEKGLELKRVGIYVKIISRKVLKTENVYDIGLEGDHNFIIKDGLIASN

SEQ ID NO: 411 - protein, 137 aa, Trichodesmium erythraeum
CLTYETEIMTVEYGPLPIGKIVEYRIECTVYTVDKNGYIYTQPIAQWHNRGMQEVYEYSLEDGTVIRATPEHKFMTEDGQMLPIDEIFERNLDLKCLGTLELVKIVSRKLAKTENVYDIGVTKDHNFVLANGLIASN

SEQ ID NO: 412 - protein, 137 aa, Microcoleus sp.
CLSYDSEILTVEYGLMPIGKIVEEGIECTVYSVDSHGYLYTQPIAQWHHRGQQEVFEYDLEDGSVIRATKDHKFMTSEGQMLAIDEIFERGLELKQVKRSQPVKIVRRKSLGIQTVYDIGVERDHNFLLANGLVASN

SEQ ID NO: 413 - protein, 137 aa, Stanieria cyanosphaera
CLSYDTEILTVEYGAMPIGKIVKEQIECNVYTVNQNGFIYPQAIAQWHERGKQEIFEYTLDNGLVIRATKDHKFMTIDGQMLPIDEIFERGLELQRINDYSNVKIVSRKSLGKQPVYDIGVTKDHNFLLSNGVVASN

SEQ ID NO: 414 - protein, 137 aa, Calothrix sp.
CLSYDTEILTWEYGFLKIGEIVEKQILCSVFSVDEQGNVYTQPIAQWHNRGLQELFAYQLEDGGVIRATKDHKFMTTDGQMLAIDEIFERQLDLFQVKGLPEVKIISRKVLKTENVYDIGLEGDHNFIIKDGLIASN

SEQ ID NO: 415 - protein, 134 aa, Cyanobacterium stanieri
CLSYDTEVLTVEYGVLPIGKIVEEQIQCTVYSVDQYGFVYTQAIAQWHDRGEQEVFEYELENGATIKATKDHKMMTSDGQMLPIDQIFEQGLDLFMVSFVKIVKRRSHGIQKVYDIGVAKDHNFLLHNGLVASN

SEQ ID NO: 416 - protein, 134 aa, Cyanothece sp.
CLSYDTEILTVEYGPMPIGKIVEENINCTVYTVDPNGFVYTQAIAQWHYRGEQEIFEYYLEDGATIRATKDHKFMTMEGKMLPIDEIFENNLDLKQLTLVKIIGRQSLGVQKVYDIGVEKEHNFLLHNGLIASN

SEQ ID NO: 417 - protein, 134 aa, Cyanothece sp.
CLSYDTEILTVEYGAIPIGKVVEENIDCTVYTVDKNGFVYTQNIAQWHLRGQQEVFEYYLDDGSILRATKDHQFMTLEGEMLPIHEIFERGLELKKIKIVKIVSYRSLGKQFVYDIGVAQDHNFLLANGSIASN

SEQ ID NO: 418 - protein, 136 aa, Anabaena sp.
CLSYDTEILTVEYGFLEIGEIVEKQIECKVYTIDSNGMLYTQSIAQWHNRGQQEVYEYLLENGAIIRATKDHKFMTEAGQMLPIDEIFAQGLDLLQVGVAEVKIVSRTYVGQANVYDIGVESDHNFVIKNGFIASN

SEQ ID NO: 419 - protein, 137 aa, Aphanothece halophytica
CLSYDTEIWTVEYGAMPIGKIVEEKIECSVYTVDENGFVYTQPIAQWHPRGQQEIIEYTLEDGRKIRATKDHKMMTESGEMLPIEEIFQRELDLKVETFHEMVKIIKRQSLGRQNVYDVCVETDHNFVLANGCVASN

SEQ ID NO: 420 - protein, 137 aa, Halothece sp.
CLSYDTEIWTVEYGAMPIGKIVEEKIECSVYTVDENGFVYTQPIAQWHPRGQQEIIEYTLEDGRKIRATKDHKMMTESGEMLPIEEIFQRELDLKVETFHEMVKIIKRQSLGRQNVYDIGVETDHNFVLANGCVASN

SEQ ID NO: 421 - protein, 137 aa, Cyanobacterium aponinum
CLSYDTEILTVEYGAISIGKIVEEKINCQVYSVDKNGFIYTQNIAQWHDRGSQELFEYELEDGRIIKATKDHKMMTKDGQMLAINDIFEQELELYSVDDMGVVKIVKRRSLGVQPVYDIGVEKDHNFILANGLVASN

SEQ ID NO: 422 - protein, 133 aa, unidentified
  REGION 1..133: note = Description of Unknown: Candidatus Atelocyanobacterium thalassa isolate sequence
CLSYDTKVLTVEYGPLPIGKVVQENIRCRVYTTNDQGLIYTQPIAQWHNRGKQEIFEYHLDDKTIIRATKEHQFMTVDHVMMPIDEIFEQGLELKKIKLKIIRRKSLGMHEVFDIGLEKDHNFVLSNGLIASN

SEQ ID NO: 423 - protein, 137 aa, Oscillatoria limnetica
CLSYNTEVLTVEYGPLPIGKIVDEQIHCRVYSVDENGFVYTQAIAQWHDRGYQEIFAYELADGSVIRATKDHQFMTEDGQMFPIDEIWEKGLDLKKLPTVQDVKIVRRQSLGVQNVYDIGVEKDHNFLLASGEIASN

SEQ ID NO: 424 - protein, 137 aa, unidentified
  source 1..137: note = Cyanobacterium endosymbiont of Epithemia turgida sequence
CLSYDTEVLTVEYGAIPIGRMVEESLDCTVYTVDKNGFVYTQSIQQWHSRGQQEIFEYCFEDGSIIRATKDHKFMTAEGKMSSIHDIFEQGLELKKIIPWSGAKIISCKSLGKQSVYDIGVVQDHNFLLANGVVASN

SEQ ID NO: 425 - protein, 133 aa, Synechococcus sp.
CLGYDTPVLTVEYGFMPIGKIVEEKIQCHVYSVDQNGLVFTQAIAQWHNRGQQEVWEYNLDNGDIVRATKDHKFMTIDGQMLPINQIFEQGLELKVIAVKIVSCKPLRVQTVYDIGVEKDHNFILDNGLVASN

SEQ ID NO: 426 - protein, 134 aa, Dactylococcopsis salina
CLSYDTEVLTEEYGAIPIGKIVEERMNCHVYSVDENGFIYSQPIAQWHPRGEQEVVEYTLEDGKIIRATADHKMMTETGEMLPIEQIFQQQLDLKISNQVKIINRQSLGKQTVYDIGVEKDHNFILGNGLVASN

SEQ ID NO: 427 - protein, 137 aa, Cylindrospermum stagnale
CLSYDTEILTVEYGFIPIGEIVEKRIECSVYSVDNHGNVYTQPIAQWHNRGLQEVFEYCLEDGSTIRATKDHKFMTTDKEMLPIDEIFERGLDLLRVEGLPIVKIIMRSYVGRENVYDIGVERDHNFVAKNGLIAAN

SEQ ID NO: 428 - protein, 137 aa, Synechocystis sp.
CLSFGTEILTVEYGPLPIGKIVSEEINCSVYSVDPEGRVYTQAIAQWHDRGEQEVLEYELEDGSVIRATSDHRFLTTDYQLLAIEEIFARQLDLLTLENIKQVKVIGRRSLGVQRIFDIGLPQDHNFLLANGAIAAN

SEQ ID NO: 429 - protein, 137 aa, Geitlerinema sp.
CLSYETPVMTVEYGPLPIGRIVEEQLDCTVYSVDEQGHVYTQPVAQWHHRGLQEVVEYELEDGRRLRATADHRFMTETGEMLPLAEIFERGLELRQVALRVPVKIVSRRSLGMQLVYDIGVAADHNFVLADGLIAAN

SEQ ID NO: 430 - protein, 137 aa, Synechocystis sp.
CLSFDAEILTVEYGPLSIGKIVGEEINCSVYSVDPQGRIYTQAIAQWHDRGVQEVFEYELEDGSVIRATPDHRFLTTDYELLAIEEIFARQMDLLTLTNLKLVKVVRRRSLGMHRVFDIGLAQDHNFLLANGAIAAN

SEQ ID NO: 431 - protein, 135 aa, Microcystis aeruginosa
CLGGETLILTEEYGLLPIAKIVSEEVNCTVYSVDKNGFVYSQPISQWHERGLQEVFEYTLENGQTIQATKDHKFMTNDGEMLAIDTIFERGLDLKSSDFSVKIISRQSLGRKPVYDIGVEKDHNFLLGNGLIASN

SEQ ID NO: 432 - protein, 135 aa, Microcystis aeruginosa
CLGGETLILTEEYGLLPIAKIVSEEINCTVYTVDQNGFVYSQPISQWHERGLQEVFEYTLENGQTIQATKDHKFMTSDGEMLAIDTIFERGLDLKSSDFSVKIIGRQSLGRKPVYDIGVEKDHNFLLGNGLIASN

SEQ ID NO: 433 - protein, 137 aa, Acaryochloris marina
CLSYDTPVLTLEYGWLPIGQVVQEQIECQVFSINERGHLYTQPIAQWHHRGQQEVFEYTLADGSTIQATAEHQFMTTDGQMYPVQQIFEEGLSLKQLPLPWQVKIIQRRSLGLQSVYDIGLAQDHNFVMANGWVAAN

SEQ ID NO: 434 - protein, 137 aa, Leptolyngbya sp.
CLDGETPIVTVEYGVLPIREIVEKELLCSVYSIDENGFVYTQPVEQWHQRGDRQMFEYQLDNGGVIRATPDHKFLTTEGEMVAIDEIFEKGLNLAEFAPADLVKILRRHSIGKAKTYDIGVSKNHNFLLANGLFASN

SEQ ID NO: 435 - protein, 137 aa, Synechococcus elongatus
CLAADTEVLTVEYGPIAIGKLVEENIRCQVYCCNPDGYIYSQPIGQWHQRGEQEVIEYELSDGRIIRATADHRFMTEEGEMLSLDEIFERSLELKQIPTPLLVKIVRRRSLGVQPVYDLGVATVHNFVLANGLVASN

SEQ ID NO: 436 - protein, 137 aa, Synechococcus sp.
CLSADTELYTVEYGWLPIGRLVEEQIECQVLSVNAHGHVYSQPIAQWHRRAWQEVFEYQLETGGTIKATTDHQFLTTDGQMYRIEDIFQRGLDLWQLPPDRFVKIISRCSLGIQPVYDIGVAQDHNFVIRGGLVASN

SEQ ID NO: 437 - protein, 137 aa, Thermosynechococcus elongatus
CLSGETAVMTVEYGAVPIRRLVQERLSCHVYSLDGQGHLYTQPIAQWHFQGFRPVYEYQLEDGSTICATPDHRFMTTRGQMLPIEQIFQEGLELWQVAIAPRGKIVGRRLMGWQAVYDIGLAADHNFVLANGAIAAN

SEQ ID NO: 438 - protein, 137 aa, Thermosynechococcus sp.
CLSGETAVMTVEYGAVPIRRLVQERLTCHVYSLDAQGHLYTQPIAQWHFQGFRPVYEYQLEDGSTIWATPDHRFMTTRGQMLPIEQIFQEGLELWQGPIAPSCKIVGRQLVGWQAVYDIGVARDHNFLLANGAIAAN

SEQ ID NO: 439 - protein, 137 aa, Thermosynechococcus vulcanus
CLSGETAVMTVEYGAIPIRRLVQERLICQVYSLDPQGHLYTQPIAQWHFQGFRPVYAYQLEDGSTICATPDHRFMTTSGQMLPIEQIFREGLELWQVAIAPPCKIVGRRLVGWQAVYDIGLAGDHNFLLANGAIAAN

SEQ ID NO: 440 - protein, 137 aa, Synechococcus sp.
CLAGGTPVVTVEYGVLPIQTIVEQELLCHVYSVDAQGLIYAQLIEQWHQRGDRLLYEYELENGQMIRATPDHRFLTTTGELLPIDEIFTQNLDLAAWAVPDSVKIIRRKFIGHAPTYDIGLSQDHNFLLGQGLIAAN

SEQ ID NO: 441 - protein, 136 aa, Scytonema hofmanni
CLSYDTEVLTAEYGFLPIGKIVEKAIECTVYSVDNDGNIYTQPIAQWHDRGQQEVFEYSLDDGSVIRATKDHKFMTTGGQMLPIDEIFERGLDLMRIDSLPVKILTRKSIGKQTVYDIGVERDHNFVIKNGLVASN

SEQ ID NO: 442 - protein, 136 aa, Westiella intricata
CLSYDTEILTVEYGFLPIGEIVEKRIECTVYTVDTNGYVYTQAIAQWHNRGEQEVFEYALEDGSIIRATKDHKFMTSEGQMLPIDEIFVKGLDLLQVQGLPVKIITRKFLGIQNVYDIGVEQNHNFVIKNGLVASN

SEQ ID NO: 443 - protein, 136 aa, Fischerella sp.
CLSYDTEILTVEYGFLPIGEIVEKGIECTVYTVDNNGNVYTQTIAQWHNRGQQEVFEYCLEDGSVIRATKDHKFMTTDGQMLPIDEIFARGLDLLQVKNLPVKIVTRRPLGTQNVYDIGVESDHNFVIKNGLVASN

SEQ ID NO: 444 - protein, 137 aa, Mastigocladopsis repens
CLSYDTEVLTVEYGFLPIGEIVEKSIECSVYTVDSNGNVYTQPIAQWHNRGQQEVFEYCLEDGSIIRATKDHKFMTIHGQMLPIDEIFERGLELMKIQGLPEAKIITRKSLGTQNVYDIGVERDHNFVTRDGFIASN

SEQ ID NO: 445 - protein, 137 aa, Scytonema hofmanni
CLSYNSEVLTVEYGFLPIGKIVEKGIECSVYSVDSYGKIYTQVIAQWHNRGQQEVFEYCLEDGTIIQATKDHKFMTVDGQMLPIDEIFERGLDLMQVQGLPDVKIITRKSLGTQNVYDIGVSSDHNFVMKNGLIASN

SEQ ID NO: 446 - protein, 137 aa, Anabaena sp.
CLSSDTEVLTVEYGLIPIGEIIEKRIDCSVFSVDKNGNIYTQPIAQWHDRGIQELYEYCLDDGSTIRATKDHKFMTTAGEMLPIDEIFERGLDLLKVHNLPQVKIITRNYVGKENVYDIGVERDHNFAIKNGLIASN

SEQ ID NO: 447 - protein, 137 aa, Fischerella sp.
CLSYDTEVLTVEYGFLPIGEIVEKRIECTVYTVDHNGYVYTQPIAQWHNRGYQEVFEYGLEDGSVIRATKDHKFMTSEGQMLPIDEIFARELDLLQVTGLVNVKIVTRRLLGIQNVYDIGVEQNHNFVIKNGLVASN

SEQ ID NO: 448 - protein, 137 aa, Calothrix sp.
CLSYDTEIFTVEYGFLPIGEIVEKRLECTVLTVDNHGNIYSQPIAQWHHRGQQQIYEYGLEDGSVIRATKDHKFMTTDGQMLPIDEIFERGLDLLQVTNLDNVKVITRKLADTENVYDIGVENHHNFLIKNGLVASN

SEQ ID NO: 449 - protein, 136 aa, Fischerella thermalis
CLSYETEILTVEYGFLPIGEIVEKRIECSVYTVDNNGYVCTQPIAQWHNRGYQEVFEYGLEDGSVIRATKDHKFMTIDRQMLPIDEIFARGLDLLQVTGLPVKIITRKSLGTQNVYDIGVEQNHNFVIKNGLVASN

SEQ ID NO: 450 - protein, 137 aa, unidentified
  source 1..137: note = cyanobacterium PCC 7702 Chl7702 sequence
CLSYDTEILTVEYGFLSIGEIVEKEIECTVYTVDSNGYIYTQPIAQWHEQGEQEIFEYSLEDGSTIRATKDHKFMTIEGEMLPIDQIFARQLDLMQITGLPQVKISTKKSLGKQKVYDIGVVRDHNFIIKNGFVASN

SEQ ID NO: 451 - protein, 136 aa, Fischerella sp.
CLSYDTEVLTVEYGFLPIGEIVEKRIECTVYTVDTNGYVYTQAIAQWHNRDEQEVFEYALEDGSIIRATKDHKFMTSEGQMLPIDEIFAKGLDLLQVQGLPVKIVTRKFLGIQNVYDIGVEQNHNFVIKNGLVASN

SEQ ID NO: 452 - protein, 137 aa, Fischerella muscicola
CLSYETEILTVEYGFLPIGEIVEKRIECSVYTVDNNGYVCTQTIAQWHNRGYQEVFEYGLEDGSVIRATKDHKFMTIDRQMLPIDEIFARGLDLLQVKGLPEVKIITRQSLGTQNVYDIGVEQNHNFVIKNGLVASN

SEQ ID NO: 453 - protein, 137 aa, Fischerella muscicola
CLSYDTEVLTVEYGFLPIGEIVEKTIECNVFTVDSNGYVYTQPIAQWHNRGYQEVFEYGLEDGSVIRATKDHKFMTSEGKMLPIDEIFARELDLLQVTGLINVKIVTRKFLGIQNVYDIGVEQNHNFVIKNGLVASN

SEQ ID NO: 454 - protein, 137 aa, Lyngbya aestuarii
CLSYDTEILTVEYGAIPIGKVVDEKIECTVYSVDKNGLIYTQPIAQWHNRGKQEVFEYSLEDGSTIRATKDHKFMTMDNQMLPIDEILEKGLELKQVNADSVVKIVSRKSLDSQTVYDIGVETDHNFLLANGSVASN

SEQ ID NO: 455 - protein, 135 aa, Microchaete sp.
CLSYKTQVLTVEYGLLAIGEIVEKNIECSVFSVDIHGNVYTQPIAQWHHRGQQEVFEYGLEDGSIIRATKDHKFMTTQGEMLPIDEIFARGLDLLQVKGVVKIITRKYIGKENVYDIGVEQDHNFAIKNGLIAAN

SEQ ID NO: 456 - protein, 137 aa, Leptolyngbya sp.
CLSYDTEILTVEYGALPIGKIVENQMICSVYSIDNNGYIYIQPIAQWHNRGQQEVFEYILEDGSIIRSTKDHKFMTKGGEMLPIDEIFERGLELAQVTRLEQVKIISRRSVGVQSVYDIGVKQDHNFFLRNGLIASN

SEQ ID NO: 457 - protein, 137 aa, Crocosphaera watsonii
CLSYDTEILTVEYGAMYIGKIVEENINCTVYTVDKNGFVYTQTIAQWHNRGEQEIFEYDLEDGSKIKATKDHKFMTIDGEMLPIDEIFEKNLDLKQVVSHPDVKIIGCRSLGTQKVYDIGVEKDHNFLLANGSIASN

SEQ ID NO: 458 - protein, 135 aa, Coleofasciculus chthonoplastes
CLSYDTQILTVEYGAVAIGEIVEKQIECTVYSVDENGYVYTQPIAQWHNRGEQEVFEYLLEDGATIRATKDHKFMTDEDQMLPIDQIFEQGLELKQVEVLVKIIGRKPLGTQPVYDIGVERDHNFLLFNGSVASN

SEQ ID NO: 459 - protein, 133 aa, Chroococcidiopsis sp.
CLSYDTEVLTVEYGAIPIGKIVEEKIACNVYSVDKNGFVYTQPIAQYHDRGIQEVFEYRLENGSVIRATKDHKMMTADGQMLPIDEIFKQNLDLKQLNVKIISRQSLGKQSVFDIGVAKDHNFLLANGLVASN

SEQ ID NO: 460 - protein, 132 aa, Aphanizomenon flos-aquae
CLSYDTEILTVEYGFLQIGEIVEKQIECKVYTVDSNGILYTQSIAQWHNRGQQEVYEYLLENGAIIRATKDHKFMTEEGQMLPIDEIFSQGLDLLQVVKIISRTYVGQANVYDIGVENDHNFVIKNGFIAAN

SEQ ID NO: 461 - protein, 137 aa, Raphidiopsis brookii
CLSYETEVLTLEYGFLPIGEIVDKQMVCTVFSVNDSGNVYTQPIGQWHDRGVQELYEYCLDDGSTIRATKDHKFMTTQGEMVPIDEIFHQGWELVQVSGTMNVKIVSRRYLGKADVYDIGVAKDHNFIIKNGLVASN

SEQ ID NO: 462 - protein, 134 aa, Cyanothece sp.
CLSYDTEILTVEYGPMPIGKIVEENINCSVYTVNKNGFVYTQSIAQWHHRGEQEVFEYYLEDGETIRATKDHKFMTTEGKMLPIDEIFENNLDLKKLTVVKIIERRSLGKQNVYDIGVEKDHNFLLSNNLIASN

SEQ ID NO: 463 - protein, 135 aa, Xenococcus sp.
CLSADTEVLTVEYGAISIGKIVEERIECTVYSVDANGFVYTQEIAQWHNRGEQEVFEYMLDDGSVIRATKDHKLMTIDGQMVAIDEIFSQGLELKQVLGLVKIVSRKSLGTQTVYDLGVARDHNFLLANGTVASN

SEQ ID NO: 464 - protein, 135 aa, Pleurocapsa sp.
CLSYDTEIYTVEYGALPIGKIVESRIKCTVLTVDKNGLVYSQPIVQWHDRGIQEVFEYTLDNGATIRATKDHKFMTVEGQMLPIDEIFELGLELKEIQQFVKIISRQSLGKQSVYDIGVAKDHNFLLANGMVASN

SEQ ID NO: 465 - protein, 137 aa, Cylindrospermopsis raciborskii
CLSYETEVLTLEYGFVPIGEIVNKQMVCTVFSLNDSGNVYTQPIGQWHDRGVQDLYEYCLDDGSTIRATKDHKFMTTQGEMVPIDEIFHQGWELVQVSGISKVKIVSRRYLGKADVYDIGVAKDHNFIIKNGLVASN

SEQ ID NO: 466 - protein, 129 aa, Spirulina major
CLTYDTLVLTVEYGPVPIGKLVEAQINCQVYSVDANGFIYTQAIAQWHDRGQRQVYEYTLEDGSTIRATPDHKFMTATGEMLPIDQIFEQGLDLVKIIHRRALPPQSVYDIGVERDHNFLLPSGWVASN

SEQ ID NO: 467 - protein, 131 aa, Spirulina subsalsa
CLSYDTKIITVEYGAIAIGTIVEQGLHCHVYSVDPNGFIYTQPIAQWHQRGEQEVFAYTLENGSIIQATKDHKFMTQQGKMLPIDTIFEQGLDLLQVKIIKRTSLGVRPVYDIGVIQDHNFLLENGLVASN

SEQ ID NO: 468 - protein, 135 aa, Microcystis aeruginosa
CLGGETLILTEEYGLLPIAKIVSEEINCTVYSVDKNGFIYSQPISQWHERGLQEVFEYTLENGQTIQATKDHKFMTSDGEMLAIDTIFERGLDLKSSDFSVKIISRQFLGRKPVYDIGVEKDHNFLLGNGLIASN

SEQ ID NO: 469 - protein, 130 aa, Myxosarcina sp.
CLSYDTEVLTLKYGALPIGEIVEKRINCHVYTRAESGFFYIQSIEQWHDRGEQEVFEYTLENGATIKATKDHKFMTSGGQMLPIDEIFERGLDLLVKIVSRKSLGKQPVYDLGVAKDHNFLLANGTVASN

SEQ ID NO: 470 - protein, 136 aa, Leptolyngbya sp.
CLSADTQLLTVEYGPLEIGRIVEEQIACHVYSVDANGFVYTQPIAQWHSRGEQEIFEYQLEDGRTLRATADHKFMTTTGEMGRINDIFEQGLDLKQIDLPQVKVVSRQSLGVQPVYDIGVATDHNFLLADGLVASN

SEQ ID NO: 471 - protein, 132 aa, Acaryochloris sp.
CLSYDTPVLTLEYGWLPIGQVVQEQIECQVFSINERGHLYTQPIAQWHHRGQQEVFEYTLTDGSTIQATAEHQFMTTDGQMYPIQQIFEEGLSLKQLVKITQRRSLGLQSVYDIGLAQDHNFVIANGWVAAN

SEQ ID NO: 472 - protein, 133 aa, Geminocystis herdmanii
CLSYDTEVLTVEFGAIPMGKIVEERLNCQVYSVDKNGFIYTQNIAQWHDRGVQEVFEYELEDGRIIKATKDHKMMIENCEMVEIDRIFEEGLELFEVNVKILKRRSISSQQVYDIGVEKDHNFLLANGLVASN

SEQ ID NO: 473 - protein, 133 aa, Nodosilinea nodulosa
CLSADTELLTLEYGPLTIGEIVAKRIPCHVFSVDESGYVYTQPVAQWHQRGHQEVFEYQLDDGTTIRATADHQFMTELGEMMAIDEIFQRGLELKQVEVKIISRQSLGVQPVYDIGVARDHNFLLADGQVASN

SEQ ID NO: 474 - protein, 137 aa, Rubidibacter lacunae
CLSYDTEVLTVEYGPLAIGTIVSERLACTVYTVDRSGFLYAQAISQWHERGRQDVFEYALDNGMTIRATKDHKLMTADGQMVAIDDIFTQGLTLKAIDTAAFMKIVSRKSLGVQHVYDIGVARDHNFLLANGAIASN

SEQ ID NO: 475 - protein, 136 aa, Chlorogloeopsisfritschii
CLSYDTAILTVEYGFLPIGEIVEKGIECTVYTVDSNGYIYTQPIAQWHNRGEQELFEYSLEDGSIIRATKDHKFMTIDGQMLPIDEIFARKLELMQVKGLPVKIIAKKSLGTQNVYDIGVERDHNFVIKNGLVASN

SEQ ID NO: 476 - protein, 137 aa, Richelia intracellularis
CLSYDTQILTVEHGPMSIGEIVEKCLECHVYTVNKNGNICIQTITQWHFRGEQEIFEYELEDGSFIQATKDHKFMTTTGEMLPIHEIFTNGLEILQLSKSLLVKILARKSLGTQKVYDIGVNDDHNFALSNSFIASN

SEQ ID NO: 477 - protein, 137 aa, Synechococcus sp.
CLAGDTPVVTVEYGVLPIQTIVEQELLCQVYSVDAQGLIYTQPIEQWHNRGDRLLYEYELENGQMIRATPDHKFLTTTGELLPIDEIFTQNLDLAAWAVPDSVKIIRRKFIGHAPTYDIGLSQDHNFLLGQGLIAAN

SEQ ID NO: 478 - protein, 137 aa, Synechococcus sp.
CLAGDTPVVTVEYGVLPIQTIVEQELLCHVYSVDAQGLIYTQPIEQWHQRGDRFLYEYELENGQMIRATPDHKFLTTTGKLLPIDEIFTQNLDLAAWAVPDSVKIIRRKFIGHAPTYDIGLSQDHNFLLGQGFIAAN

SEQ ID NO: 479 - protein, 137 aa, Synechococcus sp.
CLAGDTPVVTVEYGVLPIQTIVEQELLCHVYSVDAQGLIYTQPIEQWHQRGDRLLYEYELENGQMIRATPDHKFLTTTGELLPIDEIFTQNLDLAAWAVPDSVKILRRKFIGRAPTYDIGLSQDHNFLLGQGLVAAN

SEQ ID NO: 480 - protein, 129 aa, Synechococcus sp.
CLAGDTPVVTVEYGVLPIRTIVDQELLCHVYSLDPQGFIYAQPVEQWHRRGDRLLYEYELETGAVIRATPDHKFLTATGEMLPIDEIFVRNLDLVKIIRRNLIGEAATYDIGLGKDHNFLLGQGLIASN

SEQ ID NO: 481 - protein, 130 aa, Synechococcus sp.
CLAGGTPVVTVEYGVLPIQTIVEQELLCHVYSVDAQGLIYTQPIEQWHQRGDRLLYEYELENGQMIRATPDHKFLTTTGELLPIDEIFTQNLDLLVKIIRRKFIGHAPTYDIGLSQDHNFLLGQGLIAAN

SEQ ID NO: 482 - protein, 130 aa, Synechococcus sp.
CLAGDTPVVTVEYGVLPIQTIVEQELLCHVYSVDAQGLIYTQPIEQWHKRGDRLLYEYELENGQIIRATPDHKFLTTTGEMRPIDEIFAKNLSLLVKIIRRKFVGHAPTYDIGLSQDHNFLLGQGLIAAN

SEQ ID NO: 483 - protein, 134 aa, Cyanothece sp.; identical to SEQ ID NO: 417

SEQ ID NO: 484 - protein, 137 aa, Synechococcus elongatus; identical to SEQ ID NO: 435

SEQ ID NO: 485 - protein, 137 aa, Chlorogloeopsis fritschii
CLSYDTAILTVEYGFLPIGEIVEKGIECTVYTVDSNGYIYTQPIAQWHNRGEQELFEYSLEDGSIIRATKDHKFMTIDGQMLPIDEIFARKLELMQVKGLPEVKIIAKKSLGTQNVYDIGVERDHNFVIKNGLVASN

SEQ ID NO: 486 - protein, 132 aa, Cyanothece sp.
CLSYDTEILTVEYGPMPIGKIVEENINCTVYTVDPNGFVYTQAIAQWHYRGEQEIFEYYLEDGATIRATKDHKFMTMEGKMLPIDEIFENNLDLKQLVKIIGRQSLGVQKVYDIGVEKEHNFLLHNGLIASN

SEQ ID NO: 487 - protein, 132 aa, Lyngbya majuscula
CLSYDTEIITVEYGPIAIGEIVEKGIPCTVYSVDSNGYVYTQPIAQWHNRGEQEVFEYTLDDGSVIRATKDHKFMTIDGQMLPIDEIFEGGLELKQLVKIISRKSLGTQPVYDIGVKDDHNFILANGMVASN

SEQ ID NO: 488 - protein, 137 aa, unidentified
  source 1..137: note = filamentous cyanobacterium ESFC-1 sequence
CLSYDTEVLTVEYGAVPIGKLVEEKLNCSVYTVDPNGYIYTQAIAQWHDRGIQEVFEYQLEDNTIIRATKDHKFMTEDHQMLPIDEIFERGLELKKCPQPQQVKIIRRRSLGFQPVYDIGLEQDHNFLLNQGAIASN

SEQ ID NO: 489 - protein, 129 aa, Synechococcus sp.
CLAGGTPVVTVEYGVLPIQTIVEQELLCHVYSVDAQGLIYAQLIEQWHQRGDRLLYEYELENGQMIRATPDHRFLTTTGELLPIDEIFTQNLDLVKIIRRKFIGHAPTYDIGLSQDHNFLLGQGLIAAN

SEQ ID NO: 490 - protein, 132 aa, Acaryochloris marina
CLSYDTPVLTLEYGWLPIGQVVQEQIECQVFSINERGHLYTQPIAQWHHRGQQEVFEYTLADGSTIQATAEHQFMTTDGQMYPVQQIFEEGLSLKQLVKIIQRRSLGLQSVYDIGLAQDHNFVMANGWVAAN

SEQ ID NO: 491 - protein, 129 aa, Microcystis aeruginosa
CLGGETLILTEEYGLLPIAKIVSEEVNCTVYSVDKNGFVYSQPISQWHERGLQEVFEYTLENGQTIQATKDHKFMTNDGEMLAIDTIFERGLDLVKIISRQSLGRKPVYDIGVEKDHNFLLGNGLIASN

SEQ ID NO: 492 - protein, 125 aa, Anabaena circinalis
CLSYDTEILTVEYGFLEIGEIVEKQIECKVYTVDSNGILYTQPIAQWHHRGQQEVYEYLLENGAIIRATKDHKFMTEAGEMLPIDDIFTQVKIISRTYVGQANVYDIGVENDHNFVIKNGFVAAN

SEQ ID NO: 493 - protein, 125 aa, Anabaena circinalis
CLSYDTEILTVEYGFLEIGEIVEKQIECRVYTVDSNGILYTQPIAQWHYRGQQEVYEYLLENGAIIRATKDHNFMTEAGEMLPIDDIFTQIKIISRKYVGQANVYDIGVENDHNFVIKNGFVAAN

SEQ ID NO: 494 - protein, 124 aa, Cyanobacterium sp.
CLSYDTKVLTVEYGPLPIGKVVQENIRCRVYTTNDQGLIYTQPIAQWHNRGKQEIFEYHLDDKTIIRATKEHQFMTVDHVMMPIDEIFEQKIIRRKSLGMHEVFDIGLEKDHNFVLSNGLIASN

SEQ ID NO: 495 - protein, 129 aa, Planktothrix sp.
CLSYDTEVLTVEYGLIPISKIVEEKIECTVYTVNNQGYVYTQPIAQWHNRGEQEVFEYYLEDGSVIRATKDHKFMTVEGQMLPIDEIFEKELDLVKIISRKSLGTQPVYDIGVQEDHNFVLNNGLVASN

SEQ ID NO: 496 - protein, 129 aa, Planktothrix sp.
CLSYDTEILTVEYGLMPIGKIVKEKIECTVYTVNNQGYVYTQPIAQWHHRGEQEVFEYCLEDGSVIRATKDHKFMTVQGQMLPIDEIFEKELDLVKIISRKSLGTQPVYDIGVQEDHNFLLNNGLVASN

SEQ ID NO: 497 - protein, 137 aa, Fremyella diplosiphon
CLSYDTEVLTVEYGLIPIGEIVEKRLECSVYSVDINGNVYTQPIAQWHHRGQQEVFEYALEDGSIIRATKDHKFMTTDGQMLPIDEIFERGLDLLQVPHLPEVKIVTRRAIGAANVYDIGVEQDHNFAIKNGLIAAN

SEQ ID NO: 498 - protein, 129 aa, Planktothrix sp.
CLSYDTEILTVEYGLIPISKIVEEKIECTVYTVNNQGYVYTQPIAQWHNRGEQEVFEYYLEDGSVIRATKDHKFMTVDGQMLPIDEIFEKELDLVKIISRKSLGTQPVYDIGVQEDHNFVLNNGLVASN

SEQ ID NO: 499 - protein, 6 aa, synthetic construct
  source 1..6: note = Synthetic 6xHis tag
HHHHHH